European Patent Application EP 4 349 365 A1, published April 10, 2024. Title: PRETREATMENT FOR GENE THERAPY. Applicant: HANSA BIOPHARMA AB. Application EP. The sequence listing filed with the application follows.

SEQUENCE LISTING (97 sequences)

SEQ ID NO: 1 - protein, 339 aa, Streptococcus pyogenes
MRKRCYSTSAAVLAAVTLFVLSVDRGVIADSFSANQEIRYSEVTPYHVTSVWTKGVTPPANFTQGEDVFHAPYVANQGWYDITKTFNGKDDLLCGAATAGNMLHWWFDQNKDQIKRYLEEHPEKQKINFNGEQMFDVKEAIDTKNHQLDSKLFEYFKEKAFPYLSTKHLGVFPDHVIDMFINGYRLSLTNHGPTPVKEGSKDPRGGIFDAVFTRGDQSKLLTSRHDFKEKNLKEISDLIKKELTEGKALGLSHTYANVRINHVINLWGADFDSNGNLKAIYVTDSDSNASIGMKKYFVGVNSAGKVAISAKEIKEDNIGAQVLGLFTLSTGQDSWNQTN

SEQ ID NO: 2 - protein, 310 aa, Streptococcus pyogenes
DSFSANQEIRYSEVTPYHVTSVWTKGVTPPANFTQGEDVFHAPYVANQGWYDITKTFNGKDDLLCGAATAGNMLHWWFDQNKDQIKRYLEEHPEKQKINFNGEQMFDVKEAIDTKNHQLDSKLFEYFKEKAFPYLSTKHLGVFPDHVIDMFINGYRLSLTNHGPTPVKEGSKDPRGGIFDAVFTRGDQSKLLTSRHDFKEKNLKEISDLIKKELTEGKALGLSHTYANVRINHVINLWGADFDSNGNLKAIYVTDSDSNASIGMKKYFVGVNSAGKVAISAKEIKEDNIGAQVLGLFTLSTGQDSWNQTN

SEQ ID NO: 3 - protein, 349 aa, Streptococcus pyogenes
MKTIAYPNKPHSLSAGLLTAIAIFSLASSNITYADDYQRNATEAYAKEVPHQITSVWTKGVTPLTPEQFRYNNEDVIHAPYLAHQGWYDITKAFDGKDNLLCGAATAGNMLHWWFDQNKTEIEAYLSKHPEKQKIIFNNQELFDLKAAIDTKDSQTNSQLFNYFRDKAFPNLSARQLGVMPDLVLDMFINGYYLNVFKTQSTDVNRPYQDKDKRGGIFDAVFTRGDQTTLLTARHDLKNKGLNDISTIIKQELTEGRALALSHTYANVSISHVINLWGADFNAEGNLEAIYVTDSDANASIGMKKYFVGINAHGHVAISAKKIEGENIGAQVLGLFTLSSGKDIWQKLS

SEQ ID NO: 4 - protein, 315 aa, Streptococcus pyogenes
DDYQRNATEAYAKEVPHQITSVWTKGVTPLTPEQFRYNNEDVIHAPYLAHQGWYDITKAFDGKDNLLCGAATAGNMLHWWFDQNKTEIEAYLSKHPEKQKIIFNNQELFDLKAAIDTKDSQTNSQLFNYFRDKAFPNLSARQLGVMPDLVLDMFINGYYLNVFKTQSTDVNRPYQDKDKRGGIFDAVFTRGDQTTLLTARHDLKNKGLNDISTIIKQELTEGRALALSHTYANVSISHVINLWGADFNAEGNLEAIYVTDSDANASIGMKKYFVGINAHGHVAISAKKIEGENIGAQVLGLFTLSSGKDIWQKLS

SEQ ID NO: 5 - protein, 313 aa, Streptococcus pyogenes
DDYQRNATEAYAKEVPHQITSVWTKGVTPLTPEQFRYNNEDVFHAPYVANQGWYDITKAFDGKDNLLCGAATAGNMLHWWFDQNKDQIKRYLEEHPEKQKINFNGDNMFDVKKAIDTKNHQLDSKLFNYFKEKAFPGLSARRIGVFPDHVIDMFINGYRLSLTNHGPTPVKEGSKDPRGGIFDAVFTRGNQSKLLTSRHDFKNKNLNDISTIIKQELTKGKALGLSHTYANVSINHVINLWGADFNAEGNLEAIYVTDSDSNASIGMKKYFVGVNAHGHVAISAKKIEGENIGAQVLGLFTLSTGQDSWQKLS

SEQ ID NO: 6 - protein, 315 aa, Streptococcus pyogenes
DDYQRNATEAYAKEVPHQITSVWTKGVTPLTPEQFRYNNEDVIHAPYLANQGWYDITKAFDGKDNLLCGAATAGNMLHWWFDQNKTEIEAYLSKHPEKQKIIFRNQELFDLKEAIRTKDSQTNSQLFEYFRDKAFPYLSARQLGVMPDLVLDMFINGYYLNVFKTQSTDVKRPYQDKDKRGGIFDAVFTRGNQTTLLTARHDLKNKGLNDISTIIKEELTKGRALALSHTYANVSISHVINLWGADFNAEGNLEAIYVTDSDANASIGMKKYFVGINKHGHVAISAKKIEGENIGAQVLGLFTLSSGKDIWQKLN

SEQ ID NO: 7 - protein, 315 aa, Streptococcus pyogenes
DDYQRNATEAYAKEVPHQITSVWTKGVTPLTPEQFRYNNEDVIHAPYLAHQGWYDITKTFNGKDNLLCGAATAGNMLHWWFDQNKTEIEAYLSKHPEKQKIIFNNEELFDLKAAIDTKDSQTNSQLFNYFKEKAFPNLSTRQLGVMPDLVLDMFINGYYLNVFKTQSTDVNRPYQDKDKRGGIFDAVFTRGNQTTLLTARHDFKEKGLKDISTIIKQELTEGRALALSHTYANVSISHVINLWGADFDAEGNLKAIYVTDSDANASIGMKKYFVGINAHGKVAISAKKIEGENIGAQVLGLFTLSSGKDIWQQLS

SEQ ID NO: 8 - protein, 315 aa, Streptococcus pyogenes
DSFSANQEIRYSEVTPYHVTSVWTKGVTPLTPEQFRYNNEDVIHAPYLAHQGWYDITKAFDGKDNLLCGAATAGNMLHWWFDQNKTEIEAYLSKHPEKQKIIFNNQELFDLKAAIDTKDSQTNSQLFNYFRDKAFPNLSARQLGVMPDLVLDMFINGYYLNVFKTQSTDVNRPYQDKDKRGGIFDAVFTRGDQTTLLTARHDLKNKGLNDISTIIKQELTEGRALALSHTYANVSISHVINLWGADFNAEGNLEAIYVTDSDANASIGMKKYFVGINAHGHVAISAKKIEGENIGAQVLGLFTLSSGKDIWQKLS

SEQ ID NO: 9 - protein, 295 aa, Streptococcus pyogenes
SVWTKGVTPLTPEQFRYNNEDVIHAPYLAHQGWYDITKAFDGKDNLLCGAATAGNMLHWWFDQNKTEIEAYLSKHPEKQKIIFNNQELFDLKAAIDTKDSQTNSQLFNYFRDKAFPNLSARQLGVMPDLVLDMFINGYYLNVFKTQSTDVNRPYQDKDKRGGIFDAVFTRGDQTTLLTARHDLKNKGLNDISTIIKQELTEGRALALSHTYANVSISHVINLWGADFNAEGNLEAIYVTDSDANASIGMKKYFVGINAHGHVAISAKKIEGENIGAQVLGLFTLSSGKDIWQKLS

SEQ ID NO: 10 - protein, 314 aa, Streptococcus pyogenes
DDYQRNATEAYAKEVPHQITSVWTKGVTPLTPEQFTQGEDVIHAPYLAHQGWYDITKAFDGKDNLLCGAATAGNMLHWWFDQNKTEIEAYLSKHPEKQKIIFNNQELFDLKAAIDTKDSQTNSQLFNYFRDKAFPNLSARQLGVMPDLVLDMFINGYYLNVFKTQSTDVNRPYQDKDKRGGIFDAVFTRGDQTTLLTARHDLKNKGLNDISTIIKQELTEGRALALSHTYANVSISHVINLWGADFNAEGNLEAIYVTDSDANASIGMKKYFVGINAHGHVAISAKKIEGENIGAQVLGLFTLSSGKDIWQKLS

SEQ ID NO: 11 - protein, 312 aa, Streptococcus pyogenes
DDYQRNATEAYAKEVPHQITSVWTKGVTPPEQFTQGEDVIHAPYLAHQGWYDITKAFDGKDNLLCGAATAGNMLHWWFDQNKTEIEAYLSKHPEKQKIIFNNQELFDLKAAIDTKDSQTNSQLFNYFRDKAFPNLSARQLGVMPDLVLDMFINGYYLNVFKTQSTDVNRPYQDKDKRGGIFDAVFTRGDQTTLLTARHDLKNKGLNDISTIIKQELTEGRALALSHTYANVSISHVINLWGADFNAEGNLEAIYVTDSDANASIGMKKYFVGINAHGHVAISAKKIEGENIGAQVLGLFTLSSGKDIWQKLS

SEQ ID NO: 12 - protein, 313 aa, Streptococcus pyogenes
DDYQRNATEAYAKEVPHQITSVWTKGVTPPEQFRYNNEDVIHAPYLAHQGWYDITKAFDGKDNLLCGAATAGNMLHWWFDQNKTEIEAYLSKHPEKQKIIFNNQELFDLKAAIDTKDSQTNSQLFNYFRDKAFPNLSARQLGVMPDLVLDMFINGYYLNVFKTQSTDVNRPYQDKDKRGGIFDAVFTRGDQTTLLTARHDLKNKGLNDISTIIKQELTEGRALALSHTYANVSISHVINLWGADFNAEGNLEAIYVTDSDANASIGMKKYFVGINAHGHVAISAKKIEGENIGAQVLGLFTLSSGKDIWQKLS

SEQ ID NO: 13 - protein, 312 aa, Streptococcus pyogenes
DDYQRNATEAYAKEVPHQITSVWTKGVTPPEQFTQGEDVIHAPYLAHQGWYDITKAFDGKDNLLCGAATAGNMLHWWFDQNKTEIEAYLSKHPEKQKIIINNQELFDLKAAIDTKDSQTNSQLFNYFRDKAFPNLSARQLGVMPDLVLDMFINGYYLNVFKTQSTDVNRPYQDKDKRGGIFDAVFTRGDQTTLLTARHDLKNKGLNDISTIIKQELTEGRALALSHTYANVSISHVINLWGADFNAEGNLEAIYVTDSDANASIGMKKYFVGINAHGHVAISAKKIEGENIGAQVLGLFTLSSGKDIWQKLS

SEQ ID NO: 14 - protein, 312 aa, Streptococcus pyogenes
DDYQRNATEAYAKEVPHQITSVWTKGVTPPEQFTQGEDVIHAPYLAHQGWYDITKAFDGKDNLLCGAATAGNMLHWWFDQNKTEIEAYLSKHPEKQKIIFRNQELFDLKAAIDTKDSQTNSQLFNYFRDKAFPNLSARQLGVMPDLVLDMFINGYYLNVFKTQSTDVNRPYQDKDKRGGIFDAVFTRGDQTTLLTARHDLKNKGLNDISTIIKQELTEGRALALSHTYANVSISHVINLWGADFNAEGNLEAIYVTDSDANASIGMKKYFVGINAHGHVAISAKKIEGENIGAQVLGLFTLSSGKDIWQKLS

SEQ ID NO: 15 - protein, 312 aa, Streptococcus pyogenes
DDYQRNATEAYAKEVPHQITSVWTKGVTPPEQFTQGEDVIHAPYLAHQGWYDITKAFDGKDNLLCGAATAGNMLHWWFDQNKTEIEAYLSKHPEKQKIIIRNQELFDLKAAIDTKDSQTNSQLFNYFRDKAFPNLSARQLGVMPDLVLDMFINGYYLNVFKTQSTDVNRPYQDKDKRGGIFDAVFTRGDQTTLLTARHDLKNKGLNDISTIIKQELTEGRALALSHTYANVSISHVINLWGADFNAEGNLEAIYVTDSDANASIGMKKYFVGINAHGHVAISAKKIEGENIGAQVLGLFTLSSGKDIWQKLS

SEQ ID NO: 16 - protein, 312 aa, Streptococcus pyogenes
DDYQRNATEAYAKEVPHQITSVWTKGVTPPEQFTQGEDVIHAPYLANQGWYDITKAFDGKDNLLCGAATAGNMLHWWFDQNKTEIEAYLSKHPEKQKIIFRNQELFDLKEAIRTKDSQTNSQLFEYFRDKAFPYLSARQLGVMPDLVLDMFINGYYLNVFKTQSTDVKRPYQDKDKRGGIFDAVFTRGNQTTLLTARHDLKNKGLNDISTIIKEELTKGRALALSHTYANVSISHVINLWGADFNAEGNLEAIYVTDSDANASIGMKKYFVGINKHGHVAISAKKIEGENIGAQVLGLFTLSSGKDIWQKLN

SEQ ID NO: 17 - protein, 292 aa, Streptococcus pyogenes
SVWTKGVTPPEQFTQGEDVIHAPYLAHQGWYDITKAFDGKDNLLCGAATAGNMLHWWFDQNKTEIEAYLSKHPEKQKIIFRNQELFDLKAAIDTKDSQTNSQLFNYFRDKAFPNLSARQLGVMPDLVLDMFINGYYLNVFKTQSTDVNRPYQDKDKRGGIFDAVFTRGNQTTLLTARHDLKNKGLNDISTIIKQELTEGRALALSHTYANVSISHVINLWGADFNAEGNLEAIYVTDSDANASIGMKKYFVGINAHGHVAISAKKIEGENIGAQVLGLFTLSSGKDIWQKLS

SEQ ID NO: 18 - protein, 312 aa, Streptococcus pyogenes
DDYQRNATEAYAKEVPHQITSVWTKGVTPPEQFTQGEDVIHAPYLAHQGWYDITKAFDGADNLLCGAATAGNMLHWWFDQNKTEIEAYLSKHPEKQKIIFRNQELFDLKAAIDTKDSQTNSQLFNYFRDKAFPNLSARQLGVMPDLVLDMFINGYYLNVFKTQSTDVNRPYQDKDKRGGIFDAVFTRGNQTTLLTARHDLKNKGLNDISTIIKQELTEGRALALSHTYANVSISHVINLWGADFNAEGNLEAIYVTDSDANASIGMKKYFVGINAHGHVAISAKKIEGENIGAQVLGLFTLSSGKDIWQKLS

SEQ ID NO: 19 - protein, 292 aa, Streptococcus pyogenes
SVWTKGVTPPEQFTQGEDVIHAPYLAHQGWYDITKAFDGADNLLCGAATAGNMLHWWFDQNKTEIEAYLSKHPEKQKIIFRNQELFDLKAAIDTKDSQTNSQLFNYFRDKAFPNLSARQLGVMPDLVLDMFINGYYLNVFKTQSTDVNRPYQDKDKRGGIFDAVFTRGNQTTLLTARHDLKNKGLNDISTIIKQELTEGRALALSHTYANVSISHVINLWGADFNAEGNLEAIYVTDSDANASIGMKKYFVGINAHGHVAISAKKIEGENIGAQVLGLFTLSSGKDIWQKLS

SEQ ID NO: 20 - protein, 312 aa, Streptococcus pyogenes
DDYQRNATEAYAKEVPHQITSVWTKGVTPPEQFTQGEDVIHAPYLAHQGWYDITKAFDGKDNLLCGAATAGNMLHWWFDQNKTEIEAYLSKHPEKQKIIFRNQELFDLKAAIDTKDSQTNSQLFNYFRDKAFPNLSARQLGVMPDLVLDMFINGYYLNVFKTQSTDVNRPYQDKDKRGGIFDAVFTRGNQTTLLTARHDLKNKGLNDISTIIKQELTEGRALALSHTYANVSISHVINLWGADFNAEGNLEAIYVTDSDANASIGMKKYFVGINAHGHVAISAKKIEGENIGAQVLGLFTLSSGKDIWQKLS

SEQ ID NO: 21 - protein, 312 aa, Streptococcus pyogenes
DDYQRNATEAYAKEVPHQITSVWTKGVTPLTPEQFTQGEDVFHAPYVANQGWYDITKAFDGKDNLLCGAATAGNMLHWWFDQNKDQIKRYLEEHPEKQKINFNGENMFDVKKAIDTKNHQLDSKLFNYFKEKAFPYLSAKHLGVFPDHVIDMFINGYRLSLTNHGPTPVKEGSKDPRGGIFDAVFTRGNQSKLLTSRHDFKNKNLNDISTIIKQELTKGKALGLSHTYANVRINHVINLWGADFNAEGNLEAIYVTDSDSNASIGMKKYFVGVNAHGHVAISAKKIEGENIGAQVLGLFTLSTGQDSWQKLS

SEQ ID NO: 22 - protein, 312 aa, Streptococcus pyogenes
DDYQRNATEAYAKEVPHQITSVWTKGVTPLTPEQFTQGEDVFHAPYVANQGWYDITKAFDGKDNLLCGAATAGNMLHWWFDQNKDQIKRYLEEHPEKQKINFRGENMFDVKEAIRTKNHQLDSKLFEYFKEKAFPYLSAKHLGVFPDHVIDMFINGYRLSLTNHGPTPVKKGSKDPRGGIFDAVFTRGNQSKLLTSRHDFKNKNLNDISTIIKSELTNGKALGLSHTYANVRINHVINLWGADFNAEGNLEAIYVTDSDSNASIGMKKYFVGVNKHGHVAISAKKIEGENIGAQVLGLFTLSTGQDSWQKLN

SEQ ID NO: 23 - protein, 312 aa, Streptococcus pyogenes
DDYQRNATEAYAKEVPHQITSVWTKGVTPLTPEQFTQGEDVFHAPYVANQGWYDITKTFNGKDDLLCGAATAGNMLHWWFDQNKDQIKRYLEEHPEKQKINFNGEQMFDVKEAIDTKNHQLDSKLFEYFKEKAFPYLSTKHLGVFPDHVIDMFINGYRLSLTNHGPTPVKEGSKDPRGGIFDAVFTRGNQSKLLTSRHDFKEKNLKEISDLIKQELTEGKALGLSHTYANVRINHVINLWGADFDAEGNLKAIYVTDSDSNASIGMKKYFVGVNAAGKVAISAKKIEGENIGAQVLGLFTLSTGQDSWNQTS

SEQ ID NO: 24 - protein, 312 aa, Streptococcus pyogenes
DDYQRNATEAYAKEVPHQITSVWTKGVTPLTPEQFTQGEDVFHAPYVANQGWYDITKTFNGKDDLLCGAATAGNMLHWWFDQNKDQIKRYLEEHPEKQKINFRGEQMFDVKEAIRTKNHQLDSKLFEYFKEKAFPYLSTKHLGVFPDHVIDMFINGYRLSLTNHGPTPVKKGSKDPRGGIFDAVFTRGNQSKLLTSRHDFKEKNLKEISDLIKEELTKGKALGLSHTYANVRINHVINLWGADFDAEGNLKAIYVTDSDSNASIGMKKYFVGVNKAGKVAISAKKIEGENIGAQVLGLFTLSTGQDSWNQTN

SEQ ID NO: 25 - protein, 310 aa, Streptococcus pyogenes
DDYQRNATEAYAKEVPHQITSVWTKGVTPPEQFTQGEDVIHAPYVANQGWYDITKAFDGKDNLLCGAATAGNMLHWWFDQNKDQIKRYLEEHPEKQKINFRGEQMFDVKKAIDTKNHQLDSKLFNYFKEKAFPGLSARRIGVFPDHVIDMFINGYRLSLTNHGPTPVKEGSKDPRGGIFDAVFTRGNQSKLLTSRHDFKNKNLNDISTIIKQELTKGKALGLSHTYANVSINHVINLWGADFNAEGNLEAIYVTDSDSNASIGMKKYFVGVNAHGHVAISAKKIEGENIGAQVLGLFTLSTGQDSWQKLS

SEQ ID NO: 26 - protein, 320 aa, Streptococcus pyogenes
MDSFSANQEIRYSEVTPYHVTSVWTKGVTPPANFTQGEDVFHAPYVANQGWYDITKTFNGKDDLLCGAATAGNMLHWWFDQNKDQIKRYLEEHPEKQKINFNGEQMFDVKEAIDTKNHQLDSKLFEYFKEKAFPYLSTKHLGVFPDHVIDMFINGYRLSLTNHGPTPVKEGSKDPRGGIFDAVFTRGDQSKLLTSRHDFKEKNLKEISDLIKKELTEGKALGLSHTYANVRINHVINLWGADFDSNGNLKAIYVTDSDSNASIGMKKYFVGVNSAGKVAISAKEIKEDNIGAQVLGLFTLSTGQDSWNQTNGGGHHHHHH

SEQ ID NO: 27 - protein, 325 aa, Streptococcus pyogenes
MDDYQRNATEAYAKEVPHQITSVWTKGVTPLTPEQFRYNNEDVIHAPYLAHQGWYDITKAFDGKDNLLCGAATAGNMLHWWFDQNKTEIEAYLSKHPEKQKIIFNNQELFDLKAAIDTKDSQTNSQLFNYFRDKAFPNLSARQLGVMPDLVLDMFINGYYLNVFKTQSTDVNRPYQDKDKRGGIFDAVFTRGDQTTLLTARHDLKNKGLNDISTIIKQELTEGRALALSHTYANVSISHVINLWGADFNAEGNLEAIYVTDSDANASIGMKKYFVGINAHGHVAISAKKIEGENIGAQVLGLFTLSSGKDIWQKLSGGGHHHHHH

SEQ ID NO: 28 - protein, 323 aa, Streptococcus pyogenes
MDDYQRNATEAYAKEVPHQITSVWTKGVTPLTPEQFRYNNEDVFHAPYVANQGWYDITKAFDGKDNLLCGAATAGNMLHWWFDQNKDQIKRYLEEHPEKQKINFNGDNMFDVKKAIDTKNHQLDSKLFNYFKEKAFPGLSARRIGVFPDHVIDMFINGYRLSLTNHGPTPVKEGSKDPRGGIFDAVFTRGNQSKLLTSRHDFKNKNLNDISTIIKQELTKGKALGLSHTYANVSINHVINLWGADFNAEGNLEAIYVTDSDSNASIGMKKYFVGVNAHGHVAISAKKIEGENIGAQVLGLFTLSTGQDSWQKLSGGGHHHHHH

SEQ ID NO: 29 - protein, 11 aa, Streptococcus pyogenes
PLTPEQFRYNN

SEQ ID NO: 30 - protein, 8 aa, Streptococcus pyogenes
PPANFTQG

SEQ ID NO: 31 - protein, 20 aa, Streptococcus pyogenes
DDYQRNATEAYAKEVPHQIT

SEQ ID NO: 32 - protein, 20 aa, Streptococcus pyogenes
DSFSANQEIRYSEVTPYHVT

SEQ ID NO: 33 - DNA, 963 bp, Streptococcus pyogenes
  source 1..963: mol_type = unassigned DNA
atggatagtttttctgctaatcaagagattagatattcggaagtaacaccttatcacgttacttccgtttggaccaaaggagttactcctccagcaaacttcactcaaggtgaagatgtttttcacgctccttatgttgctaaccaaggatggtatgatattaccaaaacattcaatggaaaagacgatcttctttgcggggctgccacagcagggaatatgcttcactggtggttcgatcaaaacaaagaccaaattaaacgttatttggaagagcatccagaaaagcaaaaaataaacttcaatggcgaacagatgtttgacgtaaaagaagctatcgacactaaaaaccaccagctagatagtaaattatttgaatattttaaagaaaaagctttcccttatctatctactaaacacctaggagttttccctgatcatgtaattgatatgttcattaacggctaccgccttagtctaactaaccacggtccaacgccagtaaaagaaggtagtaaagatccccgaggtggtatttttgacgccgtatttacaagaggtgatcaaagtaagctattgacaagtcgtcatgattttaaagaaaaaaatctcaaagaaatcagtgatctcattaagaaagagttaaccgaaggcaaggctctaggcctatcacacacctacgctaacgtacgcatcaaccatgttataaacctgtggggagctgactttgattctaacgggaaccttaaagctatttatgtaacagactctgatagtaatgcatctattggtatgaagaaatactttgttggtgttaattccgctggaaaagtagctatttctgctaaagaaataaaagaagataatataggtgctcaagtactagggttatttacactttcaacagggcaagatagttggaatcagaccaatggcggtggccatcatcaccatcaccactaa

SEQ ID NO: 34 - DNA, 978 bp, Streptococcus pyogenes
  source 1..978: mol_type = unassigned DNA
atggacgattaccaaaggaatgctacggaagcttatgccaaagaagtaccacatcagatcacttctgtatggaccaaaggtgttacaccactaacacccgagcagtttcgatataataacgaagatgtgatccatgcgccatatcttgctcatcaaggctggtacgatatcaccaaggccttcgatgggaaggataatctcttgtgtggcgcagcaacggcaggtaatatgctgcattggtggtttgatcaaaataaaacagagattgaagcctatttaagtaaacaccctgaaaagcaaaaaatcatttttaacaaccaagagctatttgatttgaaagctgctatcgataccaaggacagtcaaaccaatagtcagctttttaattattttagagataaagcctttccaaatctatcagcacgtcaactcggggttatgcctgatcttgttctagatatgtttatcaatggttactacttaaatgtgtttaaaacacagtctactgatgtcaatcgaccttatcaggacaaggacaaacgaggtggtattttcgatgctgttttcaccagaggagatcagacaacgctcttgacagctcgtcatgatttaaaaaataaaggactaaatgacatcagcaccattatcaagcaagaactgactgaaggaagagcccttgctttatcacatacctacgccaatgttagcattagccatgtgattaacttgtggggagctgattttaatgctgaaggaaaccttgaggccatctatgtcacagactcagatgctaatgcgtctattggtatgaaaaaatattttgtcggcattaatgctcatggacatgtcgccatttctgccaagaaaatagaaggagaaaacattggcgctcaagtattaggcttatttacgctttccagtggcaaggacatttggcagaaactgagcggcggtggccatcatcaccatcaccactaa

SEQ ID NO: 35 - DNA, 972 bp, Streptococcus pyogenes
  source 1..972: mol_type = unassigned DNA
atggatgattatcagcgcaacgcgaccgaagcgtatgcgaaagaagtgccgcatcagattaccagcgtgtggaccaaaggcgtgaccccgctgaccccggaacagtttcgctataacaacgaagatgtgtttcatgcgccgtatgtggcgaaccagggctggtatgatattaccaaagcgtttgatggcaaagataacctgctgtgcggcgcggcgaccgcgggcaacatgctgcattggtggtttgatcagaacaaagatcagattaaacgctatctggaagaacatccggaaaaacagaaaattaactttaacggcgataacatgtttgatgtgaaaaaagcgattgataccaaaaaccatcagctggatagcaaactgtttaactattttaaagaaaaagcgtttccgggcctgagcgcgcgccgcattggcgtgtttccggatcatgtgattgatatgtttattaacggctatcgcctgagcctgaccaaccatggcccgaccccggtgaaagaaggcagcaaagatccgcgcggcggcatttttgatgcggtgtttacccgcggcaaccagagcaaactgctgaccagccgccatgattttaaaaacaaaaacctgaacgatattagcaccattattaaacaggaactgaccaaaggcaaagcgctgggcctgagccatacctatgcgaacgtgagcattaaccatgtgattaacctgtggggcgcggattttaacgcggaaggcaacctggaagcgatttatgtgaccgatagcgatagcaacgcgagcattggcatgaaaaaatattttgtgggcgtgaacgcgcatggccatgtggcgattagcgcgaaaaaaattgaaggcgaaaacattggcgcgcaggtgctgggcctgtttaccctgagcaccggccaggatagctggcagaaactgagcggcggtggccatcatcaccatcaccactaa

SEQ ID NO: 36 - DNA, 978 bp, Streptococcus pyogenes
  source 1..978: mol_type = unassigned DNA
atggatgattatcagcgcaacgcgaccgaagcgtatgcgaaagaagtgccgcatcagattaccagcgtgtggaccaaaggcgtgaccccgctgaccccggaacagtttcgctataacaacgaagatgtgattcatgcgccgtatctggcgaaccagggctggtatgatattaccaaagcgtttgatggcaaagataacctgctgtgcggcgcggcgaccgcgggcaacatgctgcattggtggtttgatcagaacaaaaccgaaattgaagcgtatctgagcaaacatccggaaaaacagaaaattatttttcgcaaccaggaactgtttgatctgaaagaagcgattcgcaccaaagatagccagaccaacagccagctgtttgaatattttcgcgataaagcgtttccgtatctgagcgcgcgccagctgggcgtgatgccggatctggtgctggatatgtttattaacggctattatctgaacgtgtttaaaacccagagcaccgatgtgaaacgcccgtatcaggataaagataaacgcggcggcatttttgatgcggtgtttacccgcggcaaccagaccaccctgctgaccgcgcgccatgatctgaaaaacaaaggcctgaacgatattagcaccattattaaagaagaactgaccaaaggccgcgcgctggcgctgagccatacctatgcgaacgtgagcattagccatgtgattaacctgtggggcgcggattttaacgcggaaggcaacctggaagcgatttatgtgaccgatagcgatgcgaacgcgagcattggcatgaaaaaatattttgtgggcattaacaaacatggccatgtggcgattagcgcgaaaaaaattgaaggcgaaaacattggcgcgcaggtgctgggcctgtttaccctgagcagcggcaaagatatttggcagaaactgaacggcggtggccatcatcaccatcaccactaa

SEQ ID NO: 37 - DNA, 978 bp, Streptococcus pyogenes
  source 1..978: mol_type = unassigned DNA
atggatgattatcagcgcaacgcgaccgaagcgtatgcgaaagaagtgccgcatcagattaccagcgtgtggaccaaaggcgtgaccccgctgaccccggaacagtttcgctataacaacgaagatgtgattcatgcgccgtatctggcgcatcagggctggtatgatattaccaaaacctttaacggcaaagataacctgctgtgcggcgcggcgaccgcgggcaacatgctgcattggtggtttgatcagaacaaaaccgaaattgaagcgtatctgagcaaacatccggaaaaacagaaaattatttttaacaacgaagaactgtttgatctgaaagcggcgattgataccaaagatagccagaccaacagccagctgtttaactattttaaagaaaaagcgtttccgaacctgagcacccgccagctgggcgtgatgccggatctggtgctggatatgtttattaacggctattatctgaacgtgtttaaaacccagagcaccgatgtgaaccgcccgtatcaggataaagataaacgcggcggcatttttgatgcggtgtttacccgcggcaaccagaccaccctgctgaccgcgcgccatgattttaaagaaaaaggcctgaaagatattagcaccattattaaacaggaactgaccgaaggccgcgcgctggcgctgagccatacctatgcgaacgtgagcattagccatgtgattaacctgtggggcgcggattttgatgcggaaggcaacctgaaagcgatttatgtgaccgatagcgatgcgaacgcgagcattggcatgaaaaaatattttgtgggcattaacgcgcatggcaaagtggcgattagcgcgaaaaaaattgaaggcgaaaacattggcgcgcaggtgctgggcctgtttaccctgagcagcggcaaagatatttggcagcagctgagcggcggtggccatcatcaccatcaccactaa

SEQ ID NO: 38 - DNA, 978 bp, Streptococcus pyogenes
  source 1..978: mol_type = unassigned DNA
atggatagctttagcgcgaaccaggaaattcgctatagcgaagtgaccccgtatcatgtgaccagcgtgtggaccaaaggcgtgaccccgctgaccccggaacagtttcgctataacaacgaagatgtgattcatgcgccgtatctggcgcatcagggctggtatgatattaccaaagcgtttgatggcaaagataacctgctgtgcggcgcggcgaccgcgggcaacatgctgcattggtggtttgatcagaacaaaaccgaaattgaagcgtatctgagcaaacatccggaaaaacagaaaattatttttaacaaccaggaactgtttgatctgaaagcggcgattgataccaaagatagccagaccaacagccagctgtttaactattttcgcgataaagcgtttccgaacctgagcgcgcgccagctgggcgtgatgccggatctggtgctggatatgtttattaacggctattatctgaacgtgtttaaaacccagagcaccgatgtgaaccgcccgtatcaggataaagataaacgcggcggcatttttgatgcggtgtttacccgcggcgatcagaccaccctgctgaccgcgcgccatgatctgaaaaacaaaggcctgaacgatattagcaccattattaaacaggaactgaccgaaggccgcgcgctggcgctgagccatacctatgcgaacgtgagcattagccatgtgattaacctgtggggcgcggattttaacgcggaaggcaacctggaagcgatttatgtgaccgatagcgatgcgaacgcgagcattggcatgaaaaaatattttgtgggcattaacgcgcatggccatgtggcgattagcgcgaaaaaaattgaaggcgaaaacattggcgcgcaggtgctgggcctgtttaccctgagcagcggcaaagatatttggcagaaactgagcggcggtggccatcatcaccatcaccactaa

SEQ ID NO: 39 - DNA, 918 bp, Streptococcus pyogenes
  source 1..918: mol_type = unassigned DNA
atgagcgtgtggaccaaaggcgtgaccccgctgaccccggaacagtttcgctataacaacgaagatgtgattcatgcgccgtatctggcgcatcagggctggtatgatattaccaaagcgtttgatggcaaagataacctgctgtgcggcgcggcgaccgcgggcaacatgctgcattggtggtttgatcagaacaaaaccgaaattgaagcgtatctgagcaaacatccggaaaaacagaaaattatttttaacaaccaggaactgtttgatctgaaagcggcgattgataccaaagatagccagaccaacagccagctgtttaactattttcgcgataaagcgtttccgaacctgagcgcgcgccagctgggcgtgatgccggatctggtgctggatatgtttattaacggctattatctgaacgtgtttaaaacccagagcaccgatgtgaaccgcccgtatcaggataaagataaacgcggcggcatttttgatgcggtgtttacccgcggcgatcagaccaccctgctgaccgcgcgccatgatctgaaaaacaaaggcctgaacgatattagcaccattattaaacaggaactgaccgaaggccgcgcgctggcgctgagccatacctatgcgaacgtgagcattagccatgtgattaacctgtggggcgcggattttaacgcggaaggcaacctggaagcgatttatgtgaccgatagcgatgcgaacgcgagcattggcatgaaaaaatattttgtgggcattaacgcgcatggccatgtggcgattagcgcgaaaaaaattgaaggcgaaaacattggcgcgcaggtgctgggcctgtttaccctgagcagcggcaaagatatttggcagaaactgagcggcggtggccatcatcaccatcaccactaa

SEQ ID NO: 40 - DNA, 975 bp, Streptococcus pyogenes
  source 1..975: mol_type = unassigned DNA
atggacgattaccaaaggaatgctacggaagcttatgccaaagaagtaccacatcagatcacttctgtatggaccaaaggtgttacaccactaacacccgagcagtttactcaaggtgaagatgtgatccatgcgccatatcttgctcatcaaggctggtacgatatcaccaaggccttcgatgggaaggataatctcttgtgtggcgcagcaacggcaggtaatatgctgcattggtggtttgatcaaaataaaacagagattgaagcctatttaagtaaacaccctgaaaagcaaaaaatcatttttaacaaccaagagctatttgatttgaaagctgctatcgataccaaggacagtcaaaccaatagtcagctttttaattattttagagataaagcctttccaaatctatcagcacgtcaactcggggttatgcctgatcttgttctagatatgtttatcaatggttactacttaaatgtgtttaaaacacagtctactgatgtcaatcgaccttatcaggacaaggacaaacgaggtggtattttcgatgctgttttcaccagaggagatcagacaacgctcttgacagctcgtcatgatttaaaaaataaaggactaaatgacatcagcaccattatcaagcaagaactgactgaaggaagagcccttgctttatcacatacctacgccaatgttagcattagccatgtgattaacttgtggggagctgattttaatgctgaaggaaaccttgaggccatctatgtcacagactcagatgctaatgcgtctattggtatgaaaaaatattttgtcggcattaatgctcatggacatgtcgccatttctgccaagaaaatagaaggagaaaacattggcgctcaagtattaggcttatttacgctttccagtggcaaggacatttggcagaaactgagcggcggtggccatcatcaccatcaccactaa

SEQ ID NO: 41 - DNA, 969 bp, Streptococcus pyogenes
  source 1..969: mol_type = unassigned DNA
atggacgattaccaaaggaatgctacggaagcttatgccaaagaagtaccacatcagatcacttctgtatggaccaaaggtgttacaccacccgagcagtttactcaaggtgaagatgtgatccatgcgccatatcttgctcatcaaggctggtacgatatcaccaaggccttcgatgggaaggataatctcttgtgtggcgcagcaacggcaggtaatatgctgcattggtggtttgatcaaaataaaacagagattgaagcctatttaagtaaacaccctgaaaagcaaaaaatcatttttaacaaccaagagctatttgatttgaaagctgctatcgataccaaggacagtcaaaccaatagtcagctttttaattattttagagataaagcctttccaaatctatcagcacgtcaactcggggttatgcctgatcttgttctagatatgtttatcaatggttactacttaaatgtgtttaaaacacagtctactgatgtcaatcgaccttatcaggacaaggacaaacgaggtggtattttcgatgctgttttcaccagaggagatcagacaacgctcttgacagctcgtcatgatttaaaaaataaaggactaaatgacatcagcaccattatcaagcaagaactgactgaaggaagagcccttgctttatcacatacctacgccaatgttagcattagccatgtgattaacttgtggggagctgattttaatgctgaaggaaaccttgaggccatctatgtcacagactcagatgctaatgcgtctattggtatgaaaaaatattttgtcggcattaatgctcatggacatgtcgccatttctgccaagaaaatagaaggagaaaacattggcgctcaagtattaggcttatttacgctttccagtggcaaggacatttggcagaaactgagcggcggtggccatcatcaccatcaccactaa

SEQ ID NO: 42 - DNA, 972 bp, Streptococcus pyogenes
  source 1..972: mol_type = unassigned DNA
atggacgattaccaaaggaatgctacggaagcttatgccaaagaagtaccacatcagatcacttctgtatggaccaaaggtgttacaccacccgagcagtttcgatataataacgaagatgtgatccatgcgccatatcttgctcatcaaggctggtacgatatcaccaaggccttcgatgggaaggataatctcttgtgtggcgcagcaacggcaggtaatatgctgcattggtggtttgatcaaaataaaacagagattgaagcctatttaagtaaacaccctgaaaagcaaaaaatcatttttaacaaccaagagctatttgatttgaaagctgctatcgataccaaggacagtcaaaccaatagtcagctttttaattattttagagataaagcctttccaaatctatcagcacgtcaactcggggttatgcctgatcttgttctagatatgtttatcaatggttactacttaaatgtgtttaaaacacagtctactgatgtcaatcgaccttatcaggacaaggacaaacgaggtggtattttcgatgctgttttcaccagaggagatcagacaacgctcttgacagctcgtcatgatttaaaaaataaaggactaaatgacatcagcaccattatcaagcaagaactgactgaaggaagagcccttgctttatcacatacctacgccaatgttagcattagccatgtgattaacttgtggggagctgattttaatgctgaaggaaaccttgaggccatctatgtcacagactcagatgctaatgcgtctattggtatgaaaaaatattttgtcggcattaatgctcatggacatgtcgccatttctgccaagaaaatagaaggagaaaacattggcgctcaagtattaggcttatttacgctttccagtggcaaggacatttggcagaaactgagcggcggtggccatcatcaccatcaccactaa

SEQ ID NO: 43 - DNA, 969 bp, Streptococcus pyogenes
  source 1..969: mol_type = unassigned DNA
atggacgattaccaaaggaatgctacggaagcttatgccaaagaagtaccacatcagatcacttctgtatggaccaaaggtgttacaccacccgagcagtttactcaaggtgaagatgtgatccatgcgccatatcttgctcatcaaggctggtacgatatcaccaaggccttcgatgggaaggataatctcttgtgtggcgcagcaacggcaggtaatatgctgcattggtggtttgatcaaaataaaacagagattgaagcctatttaagtaaacaccctgaaaagcaaaaaatcattattaacaaccaagagctatttgatttgaaagctgctatcgataccaaggacagtcaaaccaatagtcagctttttaattattttagagataaagcctttccaaatctatcagcacgtcaactcggggttatgcctgatcttgttctagatatgtttatcaatggttactacttaaatgtgtttaaaacacagtctactgatgtcaatcgaccttatcaggacaaggacaaacgaggtggtattttcgatgctgttttcaccagaggagatcagacaacgctcttgacagctcgtcatgatttaaaaaataaaggactaaatgacatcagcaccattatcaagcaagaactgactgaaggaagagcccttgctttatcacatacctacgccaatgttagcattagccatgtgattaacttgtggggagctgattttaatgctgaaggaaaccttgaggccatctatgtcacagactcagatgctaatgcgtctattggtatgaaaaaatattttgtcggcattaatgctcatggacatgtcgccatttctgccaagaaaatagaaggagaaaacattggcgctcaagtattaggcttatttacgctttccagtggcaaggacatttggcagaaactgagcggcggtggccatcatcaccatcaccactaa

SEQ ID NO: 44 - DNA, 969 bp, Streptococcus pyogenes
  source 1..969: mol_type = unassigned DNA
atggacgattaccaaaggaatgctacggaagcttatgccaaagaagtaccacatcagatcacttctgtatggaccaaaggtgttacaccacccgagcagtttactcaaggtgaagatgtgatccatgcgccatatcttgctcatcaaggctggtacgatatcaccaaggccttcgatgggaaggataatctcttgtgtggcgcagcaacggcaggtaatatgctgcattggtggtttgatcaaaataaaacagagattgaagcctatttaagtaaacaccctgaaaagcaaaaaatcatttttcgtaaccaagagctatttgatttgaaagctgctatcgataccaaggacagtcaaaccaatagtcagctttttaattattttagagataaagcctttccaaatctatcagcacgtcaactcggggttatgcctgatcttgttctagatatgtttatcaatggttactacttaaatgtgtttaaaacacagtctactgatgtcaatcgaccttatcaggacaaggacaaacgaggtggtattttcgatgctgttttcaccagaggagatcagacaacgctcttgacagctcgtcatgatttaaaaaataaaggactaaatgacatcagcaccattatcaagcaagaactgactgaaggaagagcccttgctttatcacatacctacgccaatgttagcattagccatgtgattaacttgtggggagctgattttaatgctgaaggaaaccttgaggccatctatgtcacagactcagatgctaatgcgtctattggtatgaaaaaatattttgtcggcattaatgctcatggacatgtcgccatttctgccaagaaaatagaaggagaaaacattggcgctcaagtattaggcttatttacgctttccagtggcaaggacatttggcagaaactgagcggcggtggccatcatcaccatcaccactaa

SEQ ID NO: 45 - DNA, 969 bp, Streptococcus pyogenes
  source 1..969: mol_type = unassigned DNA
atggacgattaccaaaggaatgctacggaagcttatgccaaagaagtaccacatcagatcacttctgtatggaccaaaggtgttacaccacccgagcagtttactcaaggtgaagatgtgatccatgcgccatatcttgctcatcaaggctggtacgatatcaccaaggccttcgatgggaaggataatctcttgtgtggcgcagcaacggcaggtaatatgctgcattggtggtttgatcaaaataaaacagagattgaagcctatttaagtaaacaccctgaaaagcaaaaaatcattattcgtaaccaagagctatttgatttgaaagctgctatcgataccaaggacagtcaaaccaatagtcagctttttaattattttagagataaagcctttccaaatctatcagcacgtcaactcggggttatgcctgatcttgttctagatatgtttatcaatggttactacttaaatgtgtttaaaacacagtctactgatgtcaatcgaccttatcaggacaaggacaaacgaggtggtattttcgatgctgttttcaccagaggagatcagacaacgctcttgacagctcgtcatgatttaaaaaataaaggactaaatgacatcagcaccattatcaagcaagaactgactgaaggaagagcccttgctttatcacatacctacgccaatgttagcattagccatgtgattaacttgtggggagctgattttaatgctgaaggaaaccttgaggccatctatgtcacagactcagatgctaatgcgtctattggtatgaaaaaatattttgtcggcattaatgctcatggacatgtcgccatttctgccaagaaaatagaaggagaaaacattggcgctcaagtattaggcttatttacgctttccagtggcaaggacatttggcagaaactgagcggcggtggccatcatcaccatcaccactaa

SEQ ID NO: 46 - DNA, 969 bp, Streptococcus pyogenes
  source 1..969: mol_type = unassigned DNA
atggatgattatcagcgcaacgcgaccgaagcgtatgcgaaagaagtgccgcatcagattaccagcgtgtggaccaaaggcgtgaccccgccggaacagtttactcaaggtgaagatgtgattcatgcgccgtatctggcgaaccagggctggtatgatattaccaaagcgtttgatggcaaagataacctgctgtgcggcgcggcgaccgcgggcaacatgctgcattggtggtttgatcagaacaaaaccgaaattgaagcgtatctgagcaaacatccggaaaaacagaaaattatttttcgcaaccaggaactgtttgatctgaaagaagcgattcgcaccaaagatagccagaccaacagccagctgtttgaatattttcgcgataaagcgtttccgtatctgagcgcgcgccagctgggcgtgatgccggatctggtgctggatatgtttattaacggctattatctgaacgtgtttaaaacccagagcaccgatgtgaaacgcccgtatcaggataaagataaacgcggcggcatttttgatgcggtgtttacccgcggcaaccagaccaccctgctgaccgcgcgccatgatctgaaaaacaaaggcctgaacgatattagcaccattattaaagaagaactgaccaaaggccgcgcgctggcgctgagccatacctatgcgaacgtgagcattagccatgtgattaacctgtggggcgcggattttaacgcggaaggcaacctggaagcgatttatgtgaccgatagcgatgcgaacgcgagcattggcatgaaaaaatattttgtgggcattaacaaacatggccatgtggcgattagcgcgaaaaaaattgaaggcgaaaacattggcgcgcaggtgctgggcctgtttaccctgagcagcggcaaagatatttggcagaaactgaacggcggtggccatcatcaccatcaccactaa

SEQ ID NO: 47 - DNA, 909 bp, Streptococcus pyogenes
  source 1..909: mol_type = unassigned DNA
atgtctgtatggaccaaaggtgttacaccacccgagcagtttactcaaggtgaagatgtgatccatgcgccatatcttgctcatcaaggctggtacgatatcaccaaggccttcgatgggaaggataatctcttgtgtggcgcagcaacggcaggtaatatgctgcattggtggtttgatcaaaataaaacagagattgaagcctatttaagtaaacaccctgaaaagcaaaaaatcatttttcgtaaccaagagctatttgatttgaaagctgctatcgataccaaggacagtcaaaccaatagtcagctttttaattattttagagataaagcctttccaaatctatcagcacgtcaactcggggttatgcctgatcttgttctagatatgtttatcaatggttactacttaaatgtgtttaaaacacagtctactgatgtcaatcgaccttatcaggacaaggacaaacgaggtggtattttcgatgctgttttcaccagaggaaaccagacaacgctcttgacagctcgtcatgatttaaaaaataaaggactaaatgacatcagcaccattatcaagcaagaactgactgaaggaagagcccttgctttatcacatacctacgccaatgttagcattagccatgtgattaacttgtggggagctgattttaatgctgaaggaaaccttgaggccatctatgtcacagactcagatgctaatgcgtctattggtatgaaaaaatattttgtcggcattaatgctcatggacatgtcgccatttctgccaagaaaatagaaggagaaaacattggcgctcaagtattaggcttatttacgctttccagtggcaaggacatttggcagaaactgagcggcggtggccatcatcaccatcaccactaa

SEQ ID NO: 48 - DNA, 969 bp, Streptococcus pyogenes
  source 1..969: mol_type = unassigned DNA
atggacgattaccaaaggaatgctacggaagcttatgccaaagaagtaccacatcagatcacttctgtatggaccaaaggtgttacaccacccgagcagtttactcaaggtgaagatgtgatccatgcgccatatcttgctcatcaaggctggtacgatatcaccaaggccttcgatggggcggataatctcttgtgtggcgcagcaacggcaggtaatatgctgcattggtggtttgatcaaaataaaacagagattgaagcctatttaagtaaacaccctgaaaagcaaaaaatcatttttcgtaaccaagagctatttgatttgaaagctgctatcgataccaaggacagtcaaaccaatagtcagctttttaattattttagagataaagcctttccaaatctatcagcacgtcaactcggggttatgcctgatcttgttctagatatgtttatcaatggttactacttaaatgtgtttaaaacacagtctactgatgtcaatcgaccttatcaggacaaggacaaacgaggtggtattttcgatgctgttttcaccagaggaaatcagacaacgctcttgacagctcgtcatgatttaaaaaataaaggactaaatgacatcagcaccattatcaagcaagaactgactgaaggaagagcccttgctttatcacatacctacgccaatgttagcattagccatgtgattaacttgtggggagctgattttaatgctgaaggaaaccttgaggccatctatgtcacagactcagatgctaatgcgtctattggtatgaaaaaatattttgtcggcattaatgctcatggacatgtcgccatttctgccaagaaaatagaaggagaaaacattggcgctcaagtattaggcttatttacgctttccagtggcaaggacatttggcagaaactgagcggcggtggccatcatcaccatcaccactaa

SEQ ID NO: 49 - DNA, 909 bp, Streptococcus pyogenes
  source 1..909: mol_type = unassigned DNA
atgtctgtatggaccaaaggtgttacaccacccgagcagtttactcaaggtgaagatgtgatccatgcgccatatcttgctcatcaaggctggtacgatatcaccaaggccttcgatggggcggataatctcttgtgtggcgcagcaacggcaggtaatatgctgcattggtggtttgatcaaaataaaacagagattgaagcctatttaagtaaacaccctgaaaagcaaaaaatcatttttcgtaaccaagagctatttgatttgaaagctgctatcgataccaaggacagtcaaaccaatagtcagctttttaattattttagagataaagcctttccaaatctatcagcacgtcaactcggggttatgcctgatcttgttctagatatgtttatcaatggttactacttaaatgtgtttaaaacacagtctactgatgtcaatcgaccttatcaggacaaggacaaacgaggtggtattttcgatgctgttttcaccagaggaaatcagacaacgctcttgacagctcgtcatgatttaaaaaataaaggactaaatgacatcagcaccattatcaagcaagaactgactgaaggaagagcccttgctttatcacatacctacgccaatgttagcattagccatgtgattaacttgtggggagctgattttaatgctgaaggaaaccttgaggccatctatgtcacagactcagatgctaatgcgtctattggtatgaaaaaatattttgtcggcattaatgctcatggacatgtcgccatttctgccaagaaaatagaaggagaaaacattggcgctcaagtattaggcttatttacgctttccagtggcaaggacatttggcagaaactgagcggcggtggccatcatcaccatcaccactaa

SEQ ID NO: 50 - DNA, 969 bp, Streptococcus pyogenes
  source 1..969: mol_type = unassigned DNA
atggacgattaccaaaggaatgctacggaagcttatgccaaagaagtaccacatcagatcacttctgtatggaccaaaggtgttacaccacccgagcagtttactcaaggtgaagatgtgatccatgcgccatatcttgctcatcaaggctggtacgatatcaccaaggccttcgatgggaaggataatctcttgtgtggcgcagcaacggcaggtaatatgctgcattggtggtttgatcaaaataaaacagagattgaagcctatttaagtaaacaccctgaaaagcaaaaaatcatttttcgtaaccaagagctatttgatttgaaagctgctatcgataccaaggacagtcaaaccaatagtcagctttttaattattttagagataaagcctttccaaatctatcagcacgtcaactcggggttatgcctgatcttgttctagatatgtttatcaatggttactacttaaatgtgtttaaaacacagtctactgatgtcaatcgaccttatcaggacaaggacaaacgaggtggtattttcgatgctgttttcaccagaggaaaccagacaacgctcttgacagctcgtcatgatttaaaaaataaaggactaaatgacatcagcaccattatcaagcaagaactgactgaaggaagagcccttgctttatcacatacctacgccaatgttagcattagccatgtgattaacttgtggggagctgattttaatgctgaaggaaaccttgaggccatctatgtcacagactcagatgctaatgcgtctattggtatgaaaaaatattttgtcggcattaatgctcatggacatgtcgccatttctgccaagaaaatagaaggagaaaacattggcgctcaagtattaggcttatttacgctttccagtggcaaggacatttggcagaaactgagcggcggtggccatcatcaccatcaccactaa

SEQ ID NO: 51 - DNA, 969 bp, Streptococcus pyogenes
  source 1..969: mol_type = unassigned DNA
atggatgattatcagcgcaacgcgaccgaagcgtatgcgaaagaagtgccgcatcagattaccagcgtgtggaccaaaggcgtgaccccgctgaccccggaacagtttacccagggcgaagatgtgtttcatgcgccgtatgtggcgaaccagggctggtatgatattaccaaagcgtttgatggcaaagataacctgctgtgcggcgcggcgaccgcgggcaacatgctgcattggtggtttgatcagaacaaagatcagattaaacgctatctggaagaacatccggaaaaacagaaaattaactttaacggcgaaaacatgtttgatgtgaaaaaagcgattgataccaaaaaccatcagctggatagcaaactgtttaactattttaaagaaaaagcgtttccgtatctgagcgcgaaacatctgggcgtgtttccggatcatgtgattgatatgtttattaacggctatcgcctgagcctgaccaaccatggcccgaccccggtgaaagaaggcagcaaagatccgcgcggcggcatttttgatgcggtgtttacccgcggcaaccagagcaaactgctgaccagccgccatgattttaaaaacaaaaacctgaacgatattagcaccattattaaacaggaactgaccaaaggcaaagcgctgggcctgagccatacctatgcgaacgtgcgcattaaccatgtgattaacctgtggggcgcggattttaacgcggaaggcaacctggaagcgatttatgtgaccgatagcgatagcaacgcgagcattggcatgaaaaaatattttgtgggcgtgaacgcgcatggccatgtggcgattagcgcgaaaaaaattgaaggcgaaaacattggcgcgcaggtgctgggcctgtttaccctgagcaccggccaggatagctggcagaaactgagcggcggtggccatcatcaccatcaccactaa

SEQ ID NO: 52 - DNA, 969 bp, Streptococcus pyogenes
  source 1..969: mol_type = unassigned DNA
atggatgattatcagcgcaacgcgaccgaagcgtatgcgaaagaagtgccgcatcagattaccagcgtgtggaccaaaggcgtgaccccgctgaccccggaacagtttacccagggcgaagatgtgtttcatgcgccgtatgtggcgaaccagggctggtatgatattaccaaagcgtttgatggcaaagataacctgctgtgcggcgcggcgaccgcgggcaacatgctgcattggtggtttgatcagaacaaagatcagattaaacgctatctggaagaacatccggaaaaacagaaaattaactttcgcggcgaaaacatgtttgatgtgaaagaagcgattcgcaccaaaaaccatcagctggatagcaaactgtttgaatattttaaagaaaaagcgtttccgtatctgagcgcgaaacatctgggcgtgtttccggatcatgtgattgatatgtttattaacggctatcgcctgagcctgaccaaccatggcccgaccccggtgaaaaaaggcagcaaagatccgcgcggcggcatttttgatgcggtgtttacccgcggcaaccagagcaaactgctgaccagccgccatgattttaaaaacaaaaacctgaacgatattagcaccattattaaaagcgaactgaccaacggcaaagcgctgggcctgagccatacctatgcgaacgtgcgcattaaccatgtgattaacctgtggggcgcggattttaacgcggaaggcaacctggaagcgatttatgtgaccgatagcgatagcaacgcgagcattggcatgaaaaaatattttgtgggcgtgaacaaacatggccatgtggcgattagcgcgaaaaaaattgaaggcgaaaacattggcgcgcaggtgctgggcctgtttaccctgagcaccggccaggatagctggcagaaactgaacggcggtggccatcatcaccatcaccactaa

SEQ ID NO: 53 - DNA, 969 bp, Streptococcus pyogenes
  source 1..969: mol_type = unassigned DNA
atggatgattatcagcgcaacgcgaccgaagcgtatgcgaaagaagtgccgcatcagattaccagcgtgtggaccaaaggcgtgaccccgctgaccccggaacagtttacccagggcgaagatgtgtttcatgcgccgtatgtggcgaaccagggctggtatgatattaccaaaacctttaacggcaaagatgatctgctgtgcggcgcggcgaccgcgggcaacatgctgcattggtggtttgatcagaacaaagatcagattaaacgctatctggaagaacatccggaaaaacagaaaattaactttaacggcgaacagatgtttgatgtgaaagaagcgattgataccaaaaaccatcagctggatagcaaactgtttgaatattttaaagaaaaagcgtttccgtatctgagcaccaaacatctgggcgtgtttccggatcatgtgattgatatgtttattaacggctatcgcctgagcctgaccaaccatggcccgaccccggtgaaagaaggcagcaaagatccgcgcggcggcatttttgatgcggtgtttacccgcggcaaccagagcaaactgctgaccagccgccatgattttaaagaaaaaaacctgaaagaaattagcgatctgattaaacaggaactgaccgaaggcaaagcgctgggcctgagccatacctatgcgaacgtgcgcattaaccatgtgattaacctgtggggcgcggattttgatgcggaaggcaacctgaaagcgatttatgtgaccgatagcgatagcaacgcgagcattggcatgaaaaaatattttgtgggcgtgaacgcggcgggcaaagtggcgattagcgcgaaaaaaattgaaggcgaaaacattggcgcgcaggtgctgggcctgtttaccctgagcaccggccaggatagctggaaccagaccagcggcggtggccatcatcaccatcaccactaa

SEQ ID NO: 54 - DNA, 969 bp, Streptococcus pyogenes
  source 1..969: mol_type = unassigned DNA
atggatgattatcagcgcaacgcgaccgaagcgtatgcgaaagaagtgccgcatcagattaccagcgtgtggaccaaaggcgtgaccccgctgaccccggaacagtttacccagggcgaagatgtgtttcatgcgccgtatgtggcgaaccagggctggtatgatattaccaaaacctttaacggcaaagatgatctgctgtgcggcgcggcgaccgcgggcaacatgctgcattggtggtttgatcagaacaaagatcagattaaacgctatctggaagaacatccggaaaaacagaaaattaactttcgcggcgaacagatgtttgatgtgaaagaagcgattcgcaccaaaaaccatcagctggatagcaaactgtttgaatattttaaagaaaaagcgtttccgtatctgagcaccaaacatctgggcgtgtttccggatcatgtgattgatatgtttattaacggctatcgcctgagcctgaccaaccatggcccgaccccggtgaaaaaaggcagcaaagatccgcgcggcggcatttttgatgcggtgtttacccgcggcaaccagagcaaactgctgaccagccgccatgattttaaagaaaaaaacctgaaagaaattagcgatctgattaaagaagaactgaccaaaggcaaagcgctgggcctgagccatacctatgcgaacgtgcgcattaaccatgtgattaacctgtggggcgcggattttgatgcggaaggcaacctgaaagcgatttatgtgaccgatagcgatagcaacgcgagcattggcatgaaaaaatattttgtgggcgtgaacaaagcgggcaaagtggcgattagcgcgaaaaaaattgaaggcgaaaacattggcgcgcaggtgctgggcctgtttaccctgagcaccggccaggatagctggaaccagaccaacggcggtggccatcatcaccatcaccactaa

SEQ ID NO: 55 - DNA, 963 bp, Streptococcus pyogenes
  source 1..963: mol_type = unassigned DNA
atggatgattatcagcgcaacgcgaccgaagcgtatgcgaaagaagtgccgcatcagattaccagcgtgtggaccaaaggcgtgaccccgccggaacagtttactcaaggtgaagatgtgattcatgcgccgtatgtggcgaaccagggctggtatgatattaccaaagcgtttgatggcaaagataacctgctgtgcggcgcggcgaccgcgggcaacatgctgcattggtggtttgatcagaacaaagatcagattaaacgctatctggaagaacatccggaaaaacagaaaattaactttcgcggcgaacagatgtttgatgtgaaaaaagcgattgataccaaaaaccatcagctggatagcaaactgtttaactattttaaagaaaaagcgtttccgggcctgagcgcgcgccgcattggcgtgtttccggatcatgtgattgatatgtttattaacggctatcgcctgagcctgaccaaccatggcccgaccccggtgaaagaaggcagcaaagatccgcgcggcggcatttttgatgcggtgtttacccgcggcaaccagagcaaactgctgaccagccgccatgattttaaaaacaaaaacctgaacgatattagcaccattattaaacaggaactgaccaaaggcaaagcgctgggcctgagccatacctatgcgaacgtgagcattaaccatgtgattaacctgtggggcgcggattttaacgcggaaggcaacctggaagcgatttatgtgaccgatagcgatagcaacgcgagcattggcatgaaaaaatattttgtgggcgtgaacgcgcatggccatgtggcgattagcgcgaaaaaaattgaaggcgaaaacattggcgcgcaggtgctgggcctgtttaccctgagcaccggccaggatagctggcagaaactgagcggcggtggccatcatcaccatcaccactaa

SEQ ID NO: 56 - protein, 310 aa, Streptococcus pyogenes
DSFSANQEIRYSEVTPYHVTSVWTKGVTPPANFTQGEDVFHAPYVANQGWYDITKTFNGKDDLLCGAATAGNMLHWWFDQNKDQIKRYLEEHPEKQKINFRGEQMFDVKEAIDTKNHQLDSKLFEYFKEKAFPYLSTKHLGVFPDHVIDMFINGYRLSLTNHGPTPVKEGSKDPRGGIFDAVFTRGDQSKLLTSRHDFKEKNLKEISDLIKKELTEGKALGLSHTYANVRINHVINLWGADFDSNGNLKAIYVTDSDSNASIGMKKYFVGVNSAGKVAISAKEIKEDNIGAQVLGLFTLSTGQDSWNQTN

SEQ ID NO: 57 - protein, 310 aa, Streptococcus pyogenes
DSFSANQEIRYSEVTPYHVTSVWTKGVTPPANFTQGEDVFHAPYVANQGWYDITKTFNGKDDLLCGAATAGNMLHWWFDQNKDQIKRYLEEHPEKQKINFKGEQMFDVKEAIDTKNHQLDSKLFEYFKEKAFPYLSTKHLGVFPDHVIDMFINGYRLSLTNHGPTPVKRGSKDPRGGIFDAVFTRGNQSKLLTSRHDFKEKNLKEISDLIKKELTEGKALGLSHTYANVRINHVINLWGADFDSNGNLKAIYVTDSDSNASIGMKKYFVGVNSAGKVAISAKEIKEDNIGAQVLGLFTLSTGQDSWNQTN

SEQ ID NO: 58 - protein, 310 aa, Streptococcus pyogenes
DSFSANQEIRYSEVTPYHVTSVWTKGVTPPANFTQGEDVFHAPYVANQGWYDITKTFNGKDDLLCGAATAGNMLHWWFDQNKDQIKRYLEEHPEKQKINFRGEQMFDVKEAIDTKNHQLDSKLFEYFKEKAFPYLSTKHLGVFPDHVIDMFINGYRLSLTNHGPTPVKKGSKDPRGGIFDAVFTRGNQSKLLTSRHDFKEKNLKEISDLIKKELTEGKALGLSHTYANVRINHVINLWGADFDSNGNLKAIYVTDSDSNASIGMKKYFVGVNKAGKVAISAKEIKEDNIGAQVLGLFTLSTGQDSWNQTN

SEQ ID NO: 59 - protein, 310 aa, Streptococcus pyogenes
DSFSANQEIRYSEVTPYHVTSVWTKGVTPPANFTQGEDVFHAPYVANQGWYDITKTFNGKDDLLCGAATAGNMLHWWFDQNKDQIKRYLREHPEKQKINFNGEQMFDVKEAIDTKNHQLDSKLFEYFKEKAFPYLSTKHLGVFPDHVIDMFINGYRLSLTNHGPTPVKEGSKDPRGGIFDAVFTRGNQSKLLTSRHDFKEKNLKEISDLIKKELDEGKALGLSHTYANVRINHVINLWGADFDSNGNLKAIYVTDSDSNASIGMKKYFVGVNSAGKVAISAKEIKEDNIGAQVLGLFTLSTGQDSWNQTN

SEQ ID NO: 60 - protein, 310 aa, Streptococcus pyogenes
DSFSANQEIRYSEVTPYHVTSVWTKGVTPPANFTQGEDVFHAPYVANQGWYDITKTFNGKDDLLCGAATAGNMLHWWFDQNKDQIKRYLKEHPEKQKINFNGEQMFDVKEAIRTKNHQLDSKLFEYFKEKAFPYLSTKHLGVFPDHVIDMFINGYRLSLTNHGPTPVKEGSKDPRGGIFDAVFTRGNQSKLLTSRHDFKEKNLKEISDLIKKELEEGKALGLSHTYANVRINHVINLWGADFDSNGNLKAIYVTDSDSNASIGMKKYFVGVNKAGKVAISAKEIKEDNIGAQVLGLFTLSTGQDSWNQTN

SEQ ID NO: 61 - protein, 310 aa, Streptococcus pyogenes
DSFSANQEIRYSEVTPYHVTSVWTKGVTPPANFTQGEDVFHAPYVANQGWYDITKTFNGKDDLLCGAATAGNMLHWWFDQNKDQIERYLEEHPEKQKINFNGEQMFDVKEAIDTKNHQLDSKLFEYFKEKAFPYLSTKHLGVFPDHVIDMFINGYRLSLTNHGPTPVKEGSKDPRGGIFDAVFTRGNQSKLLTSRHDFKEKNLKEISDLIKEELTKGKALGLSHTYANVRINHVINLWGADFDSNGNLKAIYVTDSDSNASIGMKKYFVGVNSAGKVAISAKEIKEKNIGAQVLGLFTLSTGQKSWNQTN

SEQ ID NO: 62 - protein, 310 aa, Streptococcus pyogenes
DSFSANQEIRYSEVTPYHVTSVWTKGVTPPANFTQGEDVFHAPYVANQGWYDITKTFNGKDDLLCGAATAGNMLHWWFDQNKDQIKRYLKEHPEKQKINFRGEQMFDVKEAIRTKNHQLDSKLFEYFKEKAFPYLSTKHLGVFPDHVIDMFINGYRLSLTNHGPTPVKEGSKDPRGGIFDAVFTRGNQSKLLTSRHDFKEKNLKEISDLIKSELENGKALGLSHTYANVRINHVINLWGADFDSNGNLKAIYVTDSDSNASIGMKKYFVGVNKAGKVAISAKEIKEDNIGAQVLGLFTLSTGQDSWNQTN

SEQ ID NO: 63 - protein, 310 aa, Streptococcus pyogenes
DSFSANQEIRYSEVTPYHVTSVWTKGVTPPANFTQGEDVFHAPYVANQGWYDITKTFNGKDDLLCGAATAGNMLHWWFDQNKDQIKRYLKEHPEKQKINFRGEQMFDVKEAIRTKNHQLDSKLFEYFKEKAFPYLSTKHLGVFPDHVIDMFINGYRLSLTNHGPTPVKKGSKDPRGGIFDAVFTRGNQSKLLTSRHDFKEKNLKEISDLIKKELEEGKALGLSHTYANVRINHVINLWGADFDSNGNLKAIYVTDSDSNASIGMKKYFVGVNSAGKVAISAKEIKEDNIGAQVLGLFTLSTGQDSWNQTN

SEQ ID NO: 64 - protein, 310 aa, Streptococcus pyogenes
DSFSANQEIRYSEVTPYHVTSVWTKGVTPPANFTQGEDVFHAPYVANQGWYDITKTFNGKDDLLCGAATAGNMLHWWFDQNKDQIERYLEEHPEKQKINFRGEQMFDVKEAIDTKNHQLDSKLFEYFKEKAFPYLSTKHLGVFPDHVIDMFINGYRLSLTNHGPTPVKKGSKDPRGGIFDAVFTRGNQSKLLTSRHDFKEKNLKEISDLIKEELTKGKALGLSHTYANVRINHVINLWGADFDSNGNLKAIYVTDSDSNASIGMKKYFVGVNSAGKVAISAKEIKEDNIGAQVLGLFTLSTGQKSWNQTN

SEQ ID NO: 65 - protein, 306 aa, Streptococcus pyogenes
DSFSANQEIRYSEVTPYHVTSVWTKGVTPPANFTQGEDVFHAPYVANQGWYDITKTFNGKDDLLCGAATAGNMLHWWFDQNKDQIKRYLEEHPEKQKINFNGEQMFDVKEAIDTKNHQLDSKLFEYFKEKAFPYLSTKHLGVFPDHVIDMFINGYRLSLTNHGPTPVKEGSKDPRGGIFDAVFTRGDQSKLLTSRHDFKEKNLKEISDLIKKELTEGKALGLSHTYANVRINHVINLWGADFDSNGNLKAIYVTDSDSNASIGMKKYFVGVNSAGKVAISAKEIKEDNIGAQVLGLFTLSTGQDSW

SEQ ID NO: 66 - protein, 290 aa, Streptococcus pyogenes
SVWTKGVTPPANFTQGEDVFHAPYVANQGWYDITKTFNGKDDLLCGAATAGNMLHWWFDQNKDQIKRYLEEHPEKQKINFNGEQMFDVKEAIDTKNHQLDSKLFEYFKEKAFPYLSTKHLGVFPDHVIDMFINGYRLSLTNHGPTPVKEGSKDPRGGIFDAVFTRGDQSKLLTSRHDFKEKNLKEISDLIKKELTEGKALGLSHTYANVRINHVINLWGADFDSNGNLKAIYVTDSDSNASIGMKKYFVGVNSAGKVAISAKEIKEDNIGAQVLGLFTLSTGQDSWNQTN

SEQ ID NO: 67 - protein, 290 aa, Streptococcus pyogenes
SVWTKGVTPPANFTQGEDVFHAPYVANQGWYDITKTFNGKDDLLCGAATAGNMLHWWFDQNKDQIKRYLEEHPEKQKINFKGEQMFDVKEAIDTKNHQLDSKLFEYFKEKAFPYLSTKHLGVFPDHVIDMFINGYRLSLTNHGPTPVKEGSKDPRGGIFDAVFTRGNQSKLLTSRHDFKEKNLKEISDLIKKELTEGKALGLSHTYANVRINHVINLWGADFDSNGNLKAIYVTDSDSNASIGMKKYFVGVNSAGKVAISAKEIKEDNIGAQVLGLFTLSTGQDSWNQTN

SEQ ID NO: 68 - protein, 290 aa, Streptococcus pyogenes
SVWTKGVTPPANFTQGEDVFHAPYVANQGWYDITKTFNGKDDLLCGAATAGNMLHWWFDQNKDQIERYLEEHPEKQKINFKGEQMFDVKKAIDTKNHQLDSKLFEYFKEKAFPYLSTKHLGVFPDHVIDMFINGYRLSLTNHGPTPVKEGSKDPRGGIFDAVFTRGNQSKLLTSRHDFKEKNLKEISDLIKEELTKGKALGLSHTYANVRINHVINLWGADFDSNGNLKAIYVTDSDSNASIGMKKYFVGVNSAGKVAISAKEIKEDNIGAQVLGLFTLSTGQKSWNQTN

SEQ ID NO: 69 - protein, 319 aa, Streptococcus pyogenes
DDYQRNATEAYAKEVPHQITSVWTKGVTPPANFTQGEDVFHAPYVANQGWYDITKTFNGKDDLLCGAATAGNMLHWWFDQNKDQIERYLEEHPEKQKINFKGEQMFDVKKAIDTKNHQLDSKLFEYFKEKAFPYLSTKHLGVFPDHVIDMFINGYRLSLTNHGPTPVKEGSKDPRGGIFDAVFTRGNQSKLLTSRHDFKEKNLKEISDLIKEELTKGKALGLSHTYANVRINHVINLWGADFDSNGNLKAIYVTDSDSNASIGMKKYFVGVNSAGKVAISAKEIKEDNIGAQVLGLFTLSTGQKSWNQTNGGGHHHHHH

SEQ ID NO: 70 - protein, 4 aa, Streptococcus pyogenes
NQTN

SEQ ID NO: 71 - protein, 20 aa, Streptococcus pyogenes
DSFSANQEIRYSEVTPYHVT

SEQ ID NO: 72 - DNA, 963 bp, Streptococcus pyogenes; identical to SEQ ID NO: 33
  source 1..963: mol_type = unassigned DNA

SEQ ID NO: 73 - DNA, 963 bp, Streptococcus pyogenes
  source 1..963: mol_type = unassigned DNA
atggatagtttttctgctaatcaagagattagatattcggaagtaacaccttatcacgttacttccgtttggaccaaaggagttactcctccagcaaacttcactcaaggtgaagatgtttttcacgctccttatgttgctaaccaaggatggtatgatattaccaaaacattcaatggaaaagacgatcttctttgcggggctgccacagcagggaatatgcttcactggtggttcgatcaaaacaaagaccaaattaaacgttatttggaagagcatccagaaaagcaaaaaataaacttccgtggcgaacagatgtttgacgtaaaagaagctatcgacactaaaaaccaccagctagatagtaaattatttgaatattttaaagaaaaagctttcccttatctatctactaaacacctaggagttttccctgatcatgtaattgatatgttcattaacggctaccgccttagtctaactaaccacggtccaacgccagtaaaagaaggtagtaaagatccccgaggtggtatttttgacgccgtatttacaagaggtgatcaaagtaagctattgacaagtcgtcatgattttaaagaaaaaaatctcaaagaaatcagtgatctcattaagaaagagttaaccgaaggcaaggctctaggcctatcacacacctacgctaacgtacgcatcaaccatgttataaacctgtggggagctgactttgattctaacgggaaccttaaagctatttatgtaacagactctgatagtaatgcatctattggtatgaagaaatactttgttggtgttaattccgctggaaaagtagctatttctgctaaagaaataaaagaagataatataggtgctcaagtactagggttatttacactttcaacagggcaagatagttggaatcagaccaatggcggtggccatcatcaccatcaccactaa

SEQ ID NO: 74 - DNA, 963 bp, Streptococcus pyogenes
  source 1..963: mol_type = unassigned DNA
atggatagtttttctgctaatcaagagattagatattcggaagtaacaccttatcacgttacttccgtttggaccaaaggagttactcctccagcaaacttcactcaaggtgaagatgtttttcacgctccttatgttgctaaccaaggatggtatgatattaccaaaacattcaatggaaaagacgatcttctttgcggggctgccacagcagggaatatgcttcactggtggttcgatcaaaacaaagaccaaattaaacgttatttggaagagcatccagaaaagcaaaaaataaacttcaaaggcgaacagatgtttgacgtaaaagaagctatcgacactaaaaaccaccagctagatagtaaattatttgaatattttaaagaaaaagctttcccttatctatctactaaacacctaggagttttccctgatcatgtaattgatatgttcattaacggctaccgccttagtctaactaaccacggtccaacgccagtaaaacgtggtagtaaagatccccgaggtggtatttttgacgccgtatttacaagaggtaaccaaagtaagctattgacaagtcgtcatgattttaaagaaaaaaatctcaaagaaatcagtgatctcattaagaaagagttaaccgaaggcaaggctctaggcctatcacacacctacgctaacgtacgcatcaaccatgttataaacctgtggggagctgactttgattctaacgggaaccttaaagctatttatgtaacagactctgatagtaatgcatctattggtatgaagaaatactttgttggtgttaattccgctggaaaagtagctatttctgctaaagaaataaaagaagataatataggtgctcaagtactagggttatttacactttcaacagggcaagatagttggaatcagaccaatggcggtggccatcatcaccatcaccactaa

SEQ ID NO: 75 - DNA, 963 bp, Streptococcus pyogenes
  source 1..963: mol_type = unassigned DNA
atggatagtttttctgctaatcaagagattagatattcggaagtaacaccttatcacgttacttccgtttggaccaaaggagttactcctccagcaaacttcactcaaggtgaagatgtttttcacgctccttatgttgctaaccaaggatggtatgatattaccaaaacattcaatggaaaagacgatcttctttgcggggctgccacagcagggaatatgcttcactggtggttcgatcaaaacaaagaccaaattaaacgttatttggaagagcatccagaaaagcaaaaaataaacttccgtggcgaacagatgtttgacgtaaaagaagctatcgacactaaaaaccaccagctagatagtaaattatttgaatattttaaagaaaaagctttcccttatctatctactaaacacctaggagttttccctgatcatgtaattgatatgttcattaacggctaccgccttagtctaactaaccacggtccaacgccagtaaaaaaaggtagtaaagatccccgaggtggtatttttgacgccgtatttacaagaggtaaccaaagtaagctattgacaagtcgtcatgattttaaagaaaaaaatctcaaagaaatcagtgatctcattaagaaagagttaaccgaaggcaaggctctaggcctatcacacacctacgctaacgtacgcatcaaccatgttataaacctgtggggagctgactttgattctaacgggaaccttaaagctatttatgtaacagactctgatagtaatgcatctattggtatgaagaaatactttgttggtgttaataaagctggaaaagtagctatttctgctaaagaaataaaagaagataatataggtgctcaagtactagggttatttacactttcaacagggcaagatagttggaatcagaccaatggcggtggccatcatcaccatcaccactaa

SEQ ID NO: 76 - DNA, 963 bp, Streptococcus pyogenes
  source 1..963: mol_type = unassigned DNA
atggatagtttttctgctaatcaagagattagatattcggaagtaacaccttatcacgttacttccgtttggaccaaaggagttactcctccagcaaacttcactcaaggtgaagatgtttttcacgctccttatgttgctaaccaaggatggtatgatattaccaaaacattcaatggaaaagacgatcttctttgcggggctgccacagcagggaatatgcttcactggtggttcgatcaaaacaaagaccaaattaaacgttatttgcgtgagcatccagaaaagcaaaaaataaacttcaatggcgaacagatgtttgacgtaaaagaagctatcgacactaaaaaccaccagctagatagtaaattatttgaatattttaaagaaaaagctttcccttatctatctactaaacacctaggagttttccctgatcatgtaattgatatgttcattaacggctaccgccttagtctaactaaccacggtccaacgccagtaaaagaaggtagtaaagatccccgaggtggtatttttgacgccgtatttacaagaggtaaccaaagtaagctattgacaagtcgtcatgattttaaagaaaaaaatctcaaagaaatcagtgatctcattaagaaagagttagatgaaggcaaggctctaggcctatcacacacctacgctaacgtacgcatcaaccatgttataaacctgtggggagctgactttgattctaacgggaaccttaaagctatttatgtaacagactctgatagtaatgcatctattggtatgaagaaatactttgttggtgttaattccgctggaaaagtagctatttctgctaaagaaataaaagaagataatataggtgctcaagtactagggttatttacactttcaacagggcaagatagttggaatcagaccaatggcggtggccatcatcaccatcaccactaa

SEQ ID NO: 77 - DNA, 963 bp, Streptococcus pyogenes
  source 1..963: mol_type = unassigned DNA
atggatagtttttctgctaatcaagagattagatattcggaagtaacaccttatcacgttacttccgtttggaccaaaggagttactcctccagcaaacttcactcaaggtgaagatgtttttcacgctccttatgttgctaaccaaggatggtatgatattaccaaaacattcaatggaaaagacgatcttctttgcggggctgccacagcagggaatatgcttcactggtggttcgatcaaaacaaagaccaaattaaacgttatttgaaagagcatccagaaaagcaaaaaataaacttcaatggcgaacagatgtttgacgtaaaagaagctatccgtactaaaaaccaccagctagatagtaaattatttgaatattttaaagaaaaagctttcccttatctatctactaaacacctaggagttttccctgatcatgtaattgatatgttcattaacggctaccgccttagtctaactaaccacggtccaacgccagtaaaagaaggtagtaaagatccccgaggtggtatttttgacgccgtatttacaagaggtaaccaaagtaagctattgacaagtcgtcatgattttaaagaaaaaaatctcaaagaaatcagtgatctcattaagaaagagttagaagaaggcaaggctctaggcctatcacacacctacgctaacgtacgcatcaaccatgttataaacctgtggggagctgactttgattctaacgggaaccttaaagctatttatgtaacagactctgatagtaatgcatctattggtatgaagaaatactttgttggtgttaataaagctggaaaagtagctatttctgctaaagaaataaaagaagataatataggtgctcaagtactagggttatttacactttcaacagggcaagatagttggaatcagaccaatggcggtggccatcatcaccatcaccactaa

SEQ ID NO: 78 - DNA, 963 bp, Streptococcus pyogenes
  source 1..963: mol_type = unassigned DNA
atggatagtttttctgctaatcaagagattagatattcggaagtaacaccttatcacgttacttccgtttggaccaaaggagttactcctccagcaaacttcactcaaggtgaagatgtttttcacgctccttatgttgctaaccaaggatggtatgatattaccaaaacattcaatggaaaagacgatcttctttgcggggctgccacagcagggaatatgcttcactggtggttcgatcaaaacaaagaccaaattgaacgttatttggaagagcatccagaaaagcaaaaaataaacttcaatggcgaacagatgtttgacgtaaaagaagctatcgacactaaaaaccaccagctagatagtaaattatttgaatattttaaagaaaaagctttcccttatctatctactaaacacctaggagttttccctgatcatgtaattgatatgttcattaacggctaccgccttagtctaactaaccacggtccaacgccagtaaaagaaggtagtaaagatccccgaggtggtatttttgacgccgtatttacaagaggtaaccaaagtaagctattgacaagtcgtcatgattttaaagaaaaaaatctcaaagaaatcagtgatctcattaaggaagagttaaccaaaggcaaggctctaggcctatcacacacctacgctaacgtacgcatcaaccatgttataaacctgtggggagctgactttgattctaacgggaaccttaaagctatttatgtaacagactctgatagtaatgcatctattggtatgaagaaatactttgttggtgttaattccgctggaaaagtagctatttctgctaaagaaataaaagaaaaaaatataggtgctcaagtactagggttatttacactttcaacagggcaaaaaagttggaatcagaccaatggcggtggccatcatcaccatcaccactaa

SEQ ID NO: 79 - DNA, 963 bp, Streptococcus pyogenes
  source 1..963: mol_type = unassigned DNA
atggatagtttttctgctaatcaagagattagatattcggaagtaacaccttatcacgttacttccgtttggaccaaaggagttactcctccagcaaacttcactcaaggtgaagatgtttttcacgctccttatgttgctaaccaaggatggtatgatattaccaaaacattcaatggaaaagacgatcttctttgcggggctgccacagcagggaatatgcttcactggtggttcgatcaaaacaaagaccaaattaaacgttatttgaaagagcatccagaaaagcaaaaaataaacttccgtggcgaacagatgtttgacgtaaaagaagctatccgtactaaaaaccaccagctagatagtaaattatttgaatattttaaagaaaaagctttcccttatctatctactaaacacctaggagttttccctgatcatgtaattgatatgttcattaacggctaccgccttagtctaactaaccacggtccaacgccagtaaaagaaggtagtaaagatccccgaggtggtatttttgacgccgtatttacaagaggtaaccaaagtaagctattgacaagtcgtcatgattttaaagaaaaaaatctcaaagaaatcagtgatctcattaagagtgagttagaaaacggcaaggctctaggcctatcacacacctacgctaacgtacgcatcaaccatgttataaacctgtggggagctgactttgattctaacgggaaccttaaagctatttatgtaacagactctgatagtaatgcatctattggtatgaagaaatactttgttggtgttaataaagctggaaaagtagctatttctgctaaagaaataaaagaagataatataggtgctcaagtactagggttatttacactttcaacagggcaagatagttggaatcagaccaatggcggtggccatcatcaccatcaccactaa

SEQ ID NO: 80 - DNA, 963 bp, Streptococcus pyogenes
  source 1..963: mol_type = unassigned DNA
atggatagtttttctgctaatcaagagattagatattcggaagtaacaccttatcacgttacttccgtttggaccaaaggagttactcctccagcaaacttcactcaaggtgaagatgtttttcacgctccttatgttgctaaccaaggatggtatgatattaccaaaacattcaatggaaaagacgatcttctttgcggggctgccacagcagggaatatgcttcactggtggttcgatcaaaacaaagaccaaattaaacgttatttgaaagagcatccagaaaagcaaaaaataaacttccgtggcgaacagatgtttgacgtaaaagaagctatccgtactaaaaaccaccagctagatagtaaattatttgaatattttaaagaaaaagctttcccttatctatctactaaacacctaggagttttccctgatcatgtaattgatatgttcattaacggctaccgccttagtctaactaaccacggtccaacgccagtaaaaaaaggtagtaaagatccccgaggtggtatttttgacgccgtatttacaagaggtaaccaaagtaagctattgacaagtcgtcatgattttaaagaaaaaaatctcaaagaaatcagtgatctcattaagaaagagttagaagaaggcaaggctctaggcctatcacacacctacgctaacgtacgcatcaaccatgttataaacctgtggggagctgactttgattctaacgggaaccttaaagctatttatgtaacagactctgatagtaatgcatctattggtatgaagaaatactttgttggtgttaattccgctggaaaagtagctatttctgctaaagaaataaaagaagataatataggtgctcaagtactagggttatttacactttcaacagggcaagatagttggaatcagaccaatggcggtggccatcatcaccatcaccactaa

SEQ ID NO: 81 - DNA, 963 bp, Streptococcus pyogenes
  source 1..963: mol_type = unassigned DNA
atggatagtttttctgctaatcaagagattagatattcggaagtaacaccttatcacgttacttccgtttggaccaaaggagttactcctccagcaaacttcactcaaggtgaagatgtttttcacgctccttatgttgctaaccaaggatggtatgatattaccaaaacattcaatggaaaagacgatcttctttgcggggctgccacagcagggaatatgcttcactggtggttcgatcaaaacaaagaccaaattgaacgttatttggaagagcatccagaaaagcaaaaaataaacttccgtggcgaacagatgtttgacgtaaaagaagctatcgacactaaaaaccaccagctagatagtaaattatttgaatattttaaagaaaaagctttcccttatctatctactaaacacctaggagttttccctgatcatgtaattgatatgttcattaacggctaccgccttagtctaactaaccacggtccaacgccagtaaaaaaaggtagtaaagatccccgaggtggtatttttgacgccgtatttacaagaggtaaccaaagtaagctattgacaagtcgtcatgattttaaagaaaaaaatctcaaagaaatcagtgatctcattaaggaagagttaaccaaaggcaaggctctaggcctatcacacacctacgctaacgtacgcatcaaccatgttataaacctgtggggagctgactttgattctaacgggaaccttaaagctatttatgtaacagactctgatagtaatgcatctattggtatgaagaaatactttgttggtgttaattccgctggaaaagtagctatttctgctaaagaaataaaagaagataatataggtgctcaagtactagggttatttacactttcaacagggcaaaaaagttggaatcagaccaatggcggtggccatcatcaccatcaccactaa

SEQ ID NO: 82 - DNA, 957 bp, Streptococcus pyogenes
  source 1..957: mol_type = unassigned DNA
atggatagtttttctgctaatcaagagattagatattcggaagtaacaccttatcacgttacttccgtttggaccaaaggagttactcctccagcaaacttcactcaaggtgaagatgtttttcacgctccttatgttgctaaccaaggatggtatgatattaccaaaacattcaatggaaaagacgatcttctttgcggggctgccacagcagggaatatgcttcactggtggttcgatcaaaacaaagaccaaattaaacgttatttggaagagcatccagaaaagcaaaaaataaacttcaatggcgaacagatgtttgacgtaaaagaagctatcgacactaaaaaccaccagctagatagtaaattatttgaatattttaaagaaaaagctttcccttatctatctactaaacacctaggagttttccctgatcatgtaattgatatgttcattaacggctaccgccttagtctaactaaccacggtccaacgccagtaaaagaaggtagtaaagatccccgaggtggtatttttgacgccgtatttacaagaggtgatcaaagtaagctattgacaagtcgtcatgattttaaagaaaaaaatctcaaagaaatcagtgatctcattaagaaagagttaaccgaaggcaaggctctaggcctatcacacacctacgctaacgtacgcatcaaccatgttataaacctgtggggagctgactttgattctaacgggaaccttaaagctatttatgtaacagactctgatagtaatgcatctattggtatgaagaaatactttgttggtgttaattccgctggaaaagtagctatttctgctaaagaaataaaagaagataatataggtgctcaagtactagggttatttacactttcaacagggcaagatagttggggtggcggcggtggccatcatcaccatcaccactaa

SEQ ID NO: 83 - DNA, 903 bp, Streptococcus pyogenes
  source 1..903: mol_type = unassigned DNA
atgtccgtttggaccaaaggagttactcctccagcaaacttcactcaaggtgaagatgtttttcacgctccttatgttgctaaccaaggatggtatgatattaccaaaacattcaatggaaaagacgatcttctttgcggggctgccacagcagggaatatgcttcactggtggttcgatcaaaacaaagaccaaattaaacgttatttggaagagcatccagaaaagcaaaaaataaacttcaatggcgaacagatgtttgacgtaaaagaagctatcgacactaaaaaccaccagctagatagtaaattatttgaatattttaaagaaaaagctttcccttatctatctactaaacacctaggagttttccctgatcatgtaattgatatgttcattaacggctaccgccttagtctaactaaccacggtccaacgccagtaaaagaaggtagtaaagatccccgaggtggtatttttgacgccgtatttacaagaggtgatcaaagtaagctattgacaagtcgtcatgattttaaagaaaaaaatctcaaagaaatcagtgatctcattaagaaagagttaaccgaaggcaaggctctaggcctatcacacacctacgctaacgtacgcatcaaccatgttataaacctgtggggagctgactttgattctaacgggaaccttaaagctatttatgtaacagactctgatagtaatgcatctattggtatgaagaaatactttgttggtgttaattccgctggaaaagtagctatttctgctaaagaaataaaagaagataatataggtgctcaagtactagggttatttacactttcaacagggcaagatagttggaatcagaccaatggcggtggccatcatcaccatcaccactaa

SEQ ID NO: 84 - DNA, 903 bp, Streptococcus pyogenes
  source 1..903: mol_type = unassigned DNA
atgtccgtttggaccaaaggagttactcctccagcaaacttcactcaaggtgaagatgtttttcacgctccttatgttgctaaccaaggatggtatgatattaccaaaacattcaatggaaaagacgatcttctttgcggggctgccacagcagggaatatgcttcactggtggttcgatcaaaacaaagaccaaattaaacgttatttggaagagcatccagaaaagcaaaaaataaacttcaaaggcgaacagatgtttgacgtaaaagaagctatcgacactaaaaaccaccagctagatagtaaattatttgaatattttaaagaaaaagctttcccttatctatctactaaacacctaggagttttccctgatcatgtaattgatatgttcattaacggctaccgccttagtctaactaaccacggtccaacgccagtaaaagaaggtagtaaagatccccgaggtggtatttttgacgccgtatttacaagaggtaaccaaagtaagctattgacaagtcgtcatgattttaaagaaaaaaatctcaaagaaatcagtgatctcattaagaaagagttaaccgaaggcaaggctctaggcctatcacacacctacgctaacgtacgcatcaaccatgttataaacctgtggggagctgactttgattctaacgggaaccttaaagctatttatgtaacagactctgatagtaatgcatctattggtatgaagaaatactttgttggtgttaattccgctggaaaagtagctatttctgctaaagaaataaaagaagataatataggtgctcaagtactagggttatttacactttcaacagggcaagatagttggaatcagaccaatggcggtggccatcatcaccatcaccactaa

SEQ ID NO: 85 - DNA, 903 bp, Streptococcus pyogenes
  source 1..903: mol_type = unassigned DNA
atgtccgtttggaccaaaggagttactcctccagcaaacttcactcaaggtgaagatgtttttcacgctccttatgttgctaaccaaggatggtatgatattaccaaaacattcaatggaaaagacgatcttctttgcggggctgccacagcagggaatatgcttcactggtggttcgatcaaaacaaagaccaaattgaacgttatttggaagagcatccagaaaagcaaaaaataaacttcaaaggcgaacagatgtttgacgtaaaaaaagctatcgacactaaaaaccaccagctagatagtaaattatttgaatattttaaagaaaaagctttcccttatctatctactaaacacctaggagttttccctgatcatgtaattgatatgttcattaacggctaccgccttagtctaactaaccacggtccaacgccagtaaaagaaggtagtaaagatccccgaggtggtatttttgacgccgtatttacaagaggtaaccaaagtaagctattgacaagtcgtcatgattttaaagaaaaaaatctcaaagaaatcagtgatctcattaaggaagagttaaccaaaggcaaggctctaggcctatcacacacctacgctaacgtacgcatcaaccatgttataaacctgtggggagctgactttgattctaacgggaaccttaaagctatttatgtaacagactctgatagtaatgcatctattggtatgaagaaatactttgttggtgttaattccgctggaaaagtagctatttctgctaaagaaataaaagaagataatataggtgctcaagtactagggttatttacactttcaacagggcaaaaaagttggaatcagaccaatggcggtggccatcatcaccatcaccactaa

SEQ ID NO: 86 - DNA, 963 bp, Streptococcus pyogenes
  source 1..963: mol_type = unassigned DNA
atggacgattaccaaaggaatgctacggaagcttatgccaaagaagtaccacatcagatcacttccgtttggaccaaaggagttactcctccagcaaacttcactcaaggtgaagatgtttttcacgctccttatgttgctaaccaaggatggtatgatattaccaaaacattcaatggaaaagacgatcttctttgcggggctgccacagcagggaatatgcttcactggtggttcgatcaaaacaaagaccaaattgaacgttatttggaagagcatccagaaaagcaaaaaataaacttcaaaggcgaacagatgtttgacgtaaaaaaagctatcgacactaaaaaccaccagctagatagtaaattatttgaatattttaaagaaaaagctttcccttatctatctactaaacacctaggagttttccctgatcatgtaattgatatgttcattaacggctaccgccttagtctaactaaccacggtccaacgccagtaaaagaaggtagtaaagatccccgaggtggtatttttgacgccgtatttacaagaggtaaccaaagtaagctattgacaagtcgtcatgattttaaagaaaaaaatctcaaagaaatcagtgatctcattaaggaagagttaaccaaaggcaaggctctaggcctatcacacacctacgctaacgtacgcatcaaccatgttataaacctgtggggagctgactttgattctaacgggaaccttaaagctatttatgtaacagactctgatagtaatgcatctattggtatgaagaaatactttgttggtgttaattccgctggaaaagtagctatttctgctaaagaaataaaagaagataatataggtgctcaagtactagggttatttacactttcaacagggcaaaaaagttggaatcagaccaatggcggtggccatcatcaccatcaccactaa

SEQ ID NO: 87 - protein, 19 aa, Streptococcus pyogenes
SFSANQEIRYSEVTPYHVT

SEQ ID NO: 88 - protein, 19 aa, Streptococcus pyogenes
DYQRNATEAYAKEVPHQIT

SEQ ID NO: 89 - protein, 20 aa, Streptococcus pyogenes
DDYQRNATEAYAKEVPHQIT

SEQ ID NO: 90 - protein, 959 aa, Streptococcus pyogenes
EEKTVQVQKGLPSIDSLHYLSENSKKEFKEELSKAGQESQKVKEILAKAQQADKQAQELAKMKIPEKIPMKPLHGPLYGGYFRTWHDKTSDPTEKDKVNSMGELPKEVDLAFIFHDWTKDYSLFWKELATKHVPKLNKQGTRVIRTIPWRFLAGGDNSGIAEDTSKYPNTPEGNKALAKAIVDEYVYKYNLDGLDVDVEHDSIPKVDKKEDTAGVERSIQVFEEIGKLIGPKGVDKSRLFIMDSTYMADKNPLIERGAPYINLLLVQVYGSQGEKGGWEPVSNRPEKTMEERWQGYSKYIRPEQYMIGFSFYEENAQEGNLWYDINSRKDEDKANGINTDITGTRAERYARWQPKTGGVKGGIFSYAIDRDGVAHQPKKYAKQKEFKDATDNIFHSDYSVSKALKTVMLKDKSYDLIDEKDFPDKALREAVMAQVGTRKGDLERFNGTLRLDNPAIQSLEGLNKFKKLAQLDLIGLSRITKLDRSVLPANMKPGKDTLETVLETYKKDNKEEPATIPPVSLKVSGLTGLKELDLSGFDRETLAGLDAATLTSLEKVDISGNKLDLAPGTENRQIFDTMLSTISNHVGSNEQTVKFDKQKPTGHYPDTYGKTSLRLPVANEKVDLQSQLLFGTVTNQGTLINSEADYKAYQNHKIAGRSFVDSNYHYNNFKVSYENYTVKVTDSTLGTTTDKTLATDKEETYKVDFFSPADKTKAVHTAKVIVGDEKTMMVNLAEGATVIGGSADPVNARKVFDGQLGSETDNISLGWDSKQSIIFKLKEDGLIKHWRFFNDSARNPETTNKPIQEASLQIFNIKDYNLDNLLENPNKFDDEKYWITVDTYSAQGERATAFSNTLNNITSKYWRVVFDTKGDRYSSPVVPELQILGYPLPNADTIMKTVTTAKELSQQKDKFSQKMLDELKIKEMALETSLNSKIFDVTAINANAGVLKDCIEKRQLLKK

SEQ ID NO: 91 - protein, 312 aa, Streptococcus equi ssp. Zooepidemicus
DDYQRNATEAYAKEVPHQITSVWTKGVTPPEQFTQGEDVIHAPYLAHQGWYDITKAFNGKDDLLCGAATAGNMLHWWFDQNKTEIEAYLSKHPEKQKIIFRNQELFDLKAAIDTKDSQTNSQLFNYFRDKAFPNLSARQLGVMPDLVLDMFINGYYLNVFKTQSTDVNRPYQDKDKRGGIFDAVFTRGNQTTLLTARHDLKNKGLNDISTIIKQELTEGRALALSHTYANVSISHVINLWGADFNAEGNLEAIYVTDSDANASIGMKKYFVGINAHGHVAISAKKIEGENIGAQVLGLFTLSSGKDIWQKLS

SEQ ID NO: 92 - protein, 292 aa, Streptococcus equi ssp. Zooepidemicus
SVWTKGVTPPEQFTQGEDVIHAPYLAHQGWYDITKAFNGKDDLLCGAATAGNMLHWWFDQNKTEIEAYLSKHPEKQKIIFRNQELFDLKAAIDTKDSQTNSQLFNYFRDKAFPNLSARQLGVMPDLVLDMFINGYYLNVFKTQSTDVNRPYQDKDKRGGIFDAVFTRGNQTTLLTARHDLKNKGLNDISTIIKQELTEGRALALSHTYANVSISHVINLWGADFNAEGNLEAIYVTDSDANASIGMKKYFVGINAHGHVAISAKKIEGENIGAQVLGLFTLSSGKDIWQKLS

SEQ ID NO: 93 - protein, 738 aa, synthetic construct
  source 1..738: note = Spk1 protein
MAADGYLPDWLEDNLSEGIREWWDLKPGAPKPKANQQKQDNGRGLVLPGYKYLGPFNGLDKGEPVNAADAAALEHDKAYDQQLQAGDNPYLRYNHADAEFQERLQEDTSFGGNLGRAVFQAKKRVLEPLGLVESPVKTAPGKKRPVEPSPQRSPDSSTGIGKKGQQPAKKRLNFGQTGDSESVPDPQPIGEPPAAPSGVGPNTMAAGGGAPMADNNEGADGVGSSSGNWHCDSTWLGDRVITTSTRTWALPTYNNHLYKQISNGTSGGSTNDNTYFGYSTPWGYFDFNRFHCHFSPRDWQRLINNNWGFRPKRLNFKLFNIQVKEVTQNEGTKTIANNLTSTIQVFTDSEYQLPYVLGSAHQGCLPPFPADVFMIPQYGYLTLNNGSQAVGRSSFYCLEYFPSQMLRTGNNFEFSYNFEDVPFHSSYAHSQSLDRLMNPLIDQYLYYLSRTQSTGGTAGTQQLLFSQAGPNNMSAQAKNWLPGPCYRQQRVSTTLSQNNNSNFAWTGATKYHLNGRDSLVNPGVAMATHKDDEERFFPSSGVLMFGKQGAGKDNVDYSSVMLTSEEEIKTTNPVATEQYGVVADNLQQQNAAPIVGAVNSQGALPGMVWQNRDVYLQGPIWAKIPHTDGNFHPSPLMGGFGLKHPPPQILIKNTPVPADPPTTFNQAKLASFITQYSTGQVSVEIEWELQKENSKRWNPEIQYTSNYYKSTNVDFAVNTEGTYSEPRPIGTRYLTRNL

SEQ ID NO: 94 - protein, 736 aa, synthetic construct
  source 1..736: note = Spk2 protein
MAADGYLPDWLEDNLSEGIREWWALQPGAPKPKANQQHQDNARGLVLPGYKYLGPGNGLDKGEPVNAADAAALEHDKAYDQQLKAGDNPYLKYNHADAEFQERLKEDTSFGGNLGRAVFQAKKRLLEPLGLVEEAAKTAPGKKRPVDQSPQEPDSSSGVGKSGKQPARKRLNFGQTGDSESVPDPQPLGEPPAAPTSLGSNTMASGGGAPMADNNEGADGVGNSSGNWHCDSQWLGDRVITTSTRTWALPTYNNHLYKQISSQSGASNDNHYFGYSTPWGYFDFNRFHCHFSPRDWQRLINNNWGFRPKKLSFKLFNIQVKEVTQNDGTTTIANNLTSTVQVFTDSEYQLPYVLGSAHQGCLPPFPADVFMVPQYGYLTLNNGSQAVGRSSFYCLEYFPSQMLRTGNNFQFSYTFEDVPFHSSYAHSQSLDRLMNPLIDQYLYYLNRTQGTTSGTTNQSRLLFSQAGPQSMSLQARNWLPGPCYRQQRLSKTANDNNNSNFPWTAASKYHLNGRDSLVNPGPAMASHKDDEEKFFPMHGNLIFGKEGTTASNAELDNVMITDEEEIRTTNPVATEQYGTVANNLQSSNTAPTTRTVNDQGALPGMVWQDRDVYLQGPIWAKIPHTDGHFHPSPLMGGFGLKHPPPQIMIKNTPVPANPPTTFSPAKFASFITQYSTGQVSVEIEWELQKENSKRWNPEIQYTSNYNKSVNVDFTVDTNGVYSEPRPIGTRYLTRPL

SEQ ID NO: 95 - DNA, 21 bp, synthetic construct
  source 1..21: mol_type = other DNA
ggaacccctagtgatggagtt

SEQ ID NO: 96 - DNA, 16 bp, synthetic construct
  source 1..16: mol_type = other DNA
cggcctcagtgagcga

SEQ ID NO: 97 - DNA, 21 bp, synthetic construct
  source 1..21: mol_type = other DNA
cactccctctctgcgcgctcg